European Patent Specification EP 3 688 032 B1, published November 5, 2025. Title: CHIMERIC ENGULFMENT RECEPTOR MOLECULES AND METHODS OF USE. Applicant: Cero Therapeutics, Inc. Corey, Daniel Mark. Application PCT. The sequence listing filed with the application follows.

SEQUENCE LISTING (177 sequences)

SEQ ID NO: 1 - protein, 292 aa, Homo sapiens
  FcgammaRI binding domain
  sig_peptide 1...15
MWFLTTLLLWVPVDGQVDTTKAVITLQPPWVSVFQEETVTLHCEVLHLPGSSSTQWFLNGTATQTSTPSYRITSASVNDSGEYRCQRGLSGRSDPIQLEIHRGWLLLQVSSRVFTEGEPLALRCHAWKDKLVYNVLYYRNGKAFKFFHWNSNLTILKTNISHNGTYHCSGMGKHRYTSAGISVTVKELFPAPVLNASVTSPLLEGNLVTLSCETKLLLQRPGLQLYFSFYMGSKTLRGRNTSSEYQILTARREDSGLYWCEAATEDGNVLKRSPELELQVLGLQLPTPVWFH

SEQ ID NO: 2 - protein, 290 aa, Homo sapiens
  Tim1 binding domain
  sig_peptide 1...20
MHPQVVILSLILHLADSVAGSVKVGGEAGPSVTLPCHYSGAVTSMCWNRGSCSLFTCQNGIVWTNGTHVTYRKDTRYKLLGDLSRRDVSLTIENTAVSDSGVYCCRVEHRGWFNDMKITVSLEIVPPKVTTTPIVTTVPTVTTVRTSTTVPTTTTVPTTTVPTTMSIPTTTTVLTTMTVSTTTSVPTTTSIPTTTSVPVTTTVSTFVPPMPLPRQNHEPVATSPSSPQPAETHPTTLQGAIRREPTSSPLYSYTTDGNDTVTESSDGLWNNNQTQLFLEHSLLTANTTKG

SEQ ID NO: 3 - protein, 314 aa, Homo sapiens
  Tim4 binding domain
  sig_peptide 1...24
MSKEPLILWLMIEFWWLYLTPVTSETVVTEVLGHRVTLPCLYSSWSHNSNSMCWGKDQCPYSGCKEALIRTDGMRVTSRKSAKYRLQGTIPRGDVSLTILNPSESDSGVYCCRIEVPGWFNDVKINVRLNLQRASTTTHRTATTTTRRTTTTSPTTTRQMTTTPAALPTTVVTTPDLTTGTPLQMTTIAVFTTANTCLSLTPSTLPEEATGLLTPEPSKEGPILTAESETVLPSDSWSSVESTSADTVLLTSKESKVWDLPSTSHVSMWKTSDSVSSPQPGASDTAVPEQNKTTKTGQMDGIPMSMKNEMPISQ

SEQ ID NO: 4 - protein, 202 aa, Homo sapiens
  Tim3 binding domain
  sig_peptide 1...21
MFSHLPFDCVLLLLLLLLTRSSEVEYRAEVGQNAYLPCFYTPAAPGNLVPVCWGKGACPVFECGNVVLRTDERDVNYWTSRYWLNGDFRKGDVSLTIENVTLADSGIYCCRIQIPGIMNDEKFNLKLVIKPAKVTPAPTRQRDFTAAFPRMLTTRGHGPAETQTLGSLPDINLTQISTLANELRDSRLANDLRDSGATIRIG

SEQ ID NO: 5 - protein, 161 aa, Homo sapiens
  FA58C2 binding domain
LNGCANPLGLKNNSIPDKQITASSSYKTWGLHLFSWNPSYARLDKQGNFNAWVAGSYGNDQWLQVDLGSSKEVTGIITQGARNFGSVQFVASYKVAYSNDSANWTEYQDPRTGSSKIFPGNWDNHSHKKNLFETPILARYVRILPVAWHNRIALRLELLGC

SEQ ID NO: 6 - protein, 94 aa, Homo sapeins
  GAS6 binding domain
  sig_peptide 1...30
MAPSLSPGPAALRRAPQLLLLLLAAECALAALLPAREATQFLRPRQRRAFQVFEEAKQGHLERECVEELCSREEAREVFENDPETDYFYPRYLD

SEQ ID NO: 7 - protein, 87 aa, Homo sapiens
  protein S binding domain
  sig_peptide 1...24
MRVLGGRCGALLACLLLVLPVSEANFLSKQQASQVLVRKRRANSLLEETKQGNLERECIEELCNKEEAREVFENDPETDYFYPKYLV

SEQ ID NO: 8 - protein, 918 aa, Homo sapiens
  BAI1 binding domain
AAGADAGPGPEPCATLVQGKFFGYFSAAAVFPANASRCSWTLRNPDPRRYTLYMKVAKAPVPCSGPGRVRTYQFDSFLESTRTYLGVESFDEVLRLCDPSAPLAFLQASKQFLQMRRQQPPQHDGLRPRAGPPGPTDDFSVEYLVVGNRNPSRAACQMLCRWLDACLAGSRSSHPCGIMQTPCACLGGEAGGPAAGPLAPRGDVCLRDAVAGGPENCLTSLTQDRGGHGATGGWKLWSLWGECTRDCGGGLQTRTRTCLPAPGVEGGGCEGVLEEGRQCNREACGPAGRTSSRSQSLRSTDARRREELGDELQQFGFPAPQTGDPAAEEWSPWSVCSSTCGEGWQTRTRFCVSSSYSTQCSGPLREQRLCNNSAVCPVHGAWDEWSPWSLCSSTCGRGFRDRTRTCRPPQFGGNPCEGPEKQTKFCNIALCPGRAVDGNWNEWSSWSACSASCSQGRQQRTRECNGPSYGGAECQGHWVETRDCFLQQCPVDGKWQAWASWGSCSVTCGAGSQRRERVCSGPFFGGAACQGPQDEYRQCGTQRCPEPHEICDEDNFGAVIWKETPAGEVAAVRCPRNATGLILRRCELDEEGIAYWEPPTYIRCVSIDYRNIQMMTREHLAKAQRGLPGEGVSEVIQTLVEISQDGTSYSGDLLSTIDVLRNMTEIFRRAYYSPTPGDVQNFVQILSNLLAEENRDKWEEAQLAGPNAKELFRLVEDFVDVIGFRMKDLRDAYQVTDNLVLSIHKLPASGATDISFPMKGWRATGDWAKVPEDRVTVSKSVFSTGLTEADEASVFVVGTVLYRNLGSFLALQRNTTVLNSKVISVTVKPPPRSLRTPLEIEFAHMYNGTTNQTCILWDETDVPSSSAPPQLGPWSWRGCRTVPLDALRTRCLCDRLSTFAILAQLSADANMEKATLPS

SEQ ID NO: 9 - DNA, 876 bp, Homo sapiens
  misc_feature: FcgammaRI binding domain
atgtggttcctgactacgttgttgctgtgggtccctgtagacggccaagtagacacaacgaaagcagtgatcacgctccaaccgccttgggtgtctgtgttccaagaagaaacagttacactgcactgtgaggtcctccacctgcctggttcttcatctactcaatggtttctcaacggaacagcaacacaaacaagtaccccttcctacagaattacgagtgcatctgttaacgattcaggagagtataggtgccagcgagggctttcaggccggtccgaccccattcaactcgaaattcaccgcggttggcttctgctgcaagtatcctctcgggtcttcacggaaggtgaaccacttgccttgcgctgtcacgcatggaaagataagctcgtctacaacgttttgtattatcggaatggaaaggcatttaagttttttcattggaactcaaaccttacgatcctcaaaaccaatatcagtcataacggtacgtaccactgctcaggcatgggcaagcatcgctatacgtccgcagggattagcgtgacagttaaggagctcttccccgcgcctgtgctgaatgcgagcgtaacttcaccccttctggagggcaacttggtgaccctctcttgtgagacgaaacttctccttcagaggccgggcctgcaactctatttcagcttttatatgggttctaaaactcttcgaggcagaaacacgagcagcgaatatcagatactgactgcccggcgggaagacagtggcctttattggtgcgaggctgcaacagaagatggcaatgtccttaaaaggtctcccgaattggagctccaagtgcttggcttgcaactccctacacccgtatggttccac

SEQ ID NO: 10 - DNA, 870 bp, Homo sapiens
  misc_feature: Tim1 binding domain
atgcacccccaggttgttatactttcattgatcctgcatttggccgactccgtggcgggttccgtaaaagttggaggggaagctggaccaagcgtcaccttgccttgccactactctggagccgtgacgagtatgtgctggaatcgaggatcctgtagtcttttcacatgccaaaatggcatagtttggaccaatgggacgcacgtcacctaccgaaaagacactagatacaaactcctgggtgacctcagcaggagagatgtgtctctgactattgaaaacactgctgtttctgactctggagtctactgttgccgggtcgagcaccgaggatggttcaatgacatgaagatcacggtcagcttggaaatcgtcccgcccaaggtaaccactacaccaatagttactacggttcccacggtaaccacggttcgaaccagcaccacagtacccacaactacgaccgttccaaccactacagtccccacaaccatgagtatccctacgacaactacggtcctgacaaccatgaccgtcagcactaccacgagtgtgcctacgactactagcataccgacgactacttcagttccagtcaccaccacggtgagtacattcgtgcctccaatgccattgccgaggcaaaaccacgaacccgtggcgacatctccgtctagtccgcaaccagcagagacccatcccaccacgcttcagggggcaatcaggagagaacctacaagttcacccctctacagctatacaaccgatggaaacgacacagttacagaaagtagtgacggtttgtggaataacaaccaaacacaattgttcctggagcacagtctgttgacagccaacactacaaaggga

SEQ ID NO: 11 - DNA, 942 bp, Homo sapiens
  misc_feature: Tim4 binding domain
atgagtaaagagccgcttatcctgtggcttatgatagagttttggtggttgtatttgaccccggtcacgagcgaaacggtagtgactgaagtattgggtcatcgggtaaccttgccttgcttgtatagctcctggtctcataatagtaatagcatgtgctggggcaaggaccaatgcccctatagcggatgcaaggaggcgctcattcgcacagacggaatgcgggtgacatcaaggaagagtgctaagtaccggcttcagggcacaatcccacgcggcgacgtgtcactgactatccttaatccatccgagagcgactctggtgtctattgttgcaggatcgaggttccgggatggttcaatgatgtaaagatcaatgtaagactcaatctgcaacgggcatctacaaccacgcatcggacagccactactaccacaaggagaacaactactacgtcacccacgactactcgacagatgaccactacacctgcggccctgccaactacggttgtaactactccggatctgacaaccgggacaccgttgcaaatgacaaccattgcagtatttaccacggcaaacacgtgtctctctctgaccccatctactcttccggaggaggccaccgggctccttacaccggagccgtctaaggaaggcccaatcttgaccgcagagagtgagaccgtacttccgagcgattcatggtccagtgtcgagagcacatccgctgacaccgtccttcttacgtccaaagaaagtaaagtttgggacctcccgtccacgagccacgtttctatgtggaagacctcagatagcgttagctccccacagccaggagcaagcgacaccgcagtaccggagcaaaacaagacgactaagactggccagatggatggtatcccaatgtcaatgaaaaatgagatgcccatatcacaa

SEQ ID NO: 12 - DNA, 606 bp, Homo sapiens
  misc_feature: Tim3 binding domain
atgtttagccatctcccttttgattgcgtcttgttgcttcttcttctccttctgacgagatcatctgaagttgaatatcgcgcggaagtcggccaaaacgcatatctgccgtgtttttacaccccggctgcaccggggaacttggttcccgtttgttggggtaagggggcgtgtcccgtttttgagtgcggtaacgtagtgctccgaactgatgaaagagatgtaaattactggacgagccggtactggttgaatggggattttaggaagggcgacgtttcccttaccatagaaaacgtaactcttgcggattctgggatttattgttgcaggatacaaatccccggaataatgaacgatgagaaattcaatttgaagctcgtaataaaaccggcaaaagtaactccagctcccaccaggcagcgagattttacggcagcatttcccaggatgctcactactcgcggtcatggccctgccgagactcagaccctcggtagtcttcctgatatcaatctcacgcaaattagtacattggcgaatgaattgagggattcaagactcgccaatgatctgcgcgacagtggagcgactattaggataggg

SEQ ID NO: 13 - DNA, 483 bp, Homo sapiens
  misc_feature: FA58C2 binding domain
ctcaacgggtgtgctaatccccttggcctgaagaataacagcatacctgacaagcaaataacagcgtcaagttcttataaaacttgggggctgcatctgttctcctggaaccccagttacgctagactcgacaaacaaggcaattttaacgcatgggtggcaggctcttacgggaacgatcagtggctgcaagtagacttgggaagtagtaaggaggtgactgggatcattacccagggggcacgaaatttcggttccgttcagttcgttgcatcttataaggtagcgtattcaaatgactccgcgaattggaccgaatatcaggacccgcgaaccggatcaagcaagatttttccggggaattgggacaaccactctcacaaaaaaaatttgtttgaaacacctatactggcgcggtacgttagaatcctcccagttgcctggcacaaccggatagcgcttagactggaattgttggggtgc

SEQ ID NO: 14 - DNA, 282 bp, Homo sapiens
  misc_feature: Gas6 binding domain
atggctccctctttgtcaccaggacctgcggctcttaggcgagccccgcagctgctgcttctcctgctcgctgcagaatgcgctctcgctgcactcttgcccgcgagggaggcgactcagttcttgcgcccccggcagagacgagcattccaagtctttgaggaagcgaaacaaggtcatctcgagcgagaatgcgtggaggagctgtgttctagggaggaagcacgcgaagtctttgagaatgacccggaaacggactacttttacccccggtatcttgat

SEQ ID NO: 15 - DNA, 261 bp, Homo sapiens
  misc_feature: Protein S binding domain
atgcgcgtgttggggggtcgctgtggtgcgctccttgcttgtctccttttggttcttcccgtctccgaggctaatttcctgtcaaaacaacaggctagtcaagtcttggtgcgcaagaggagagctaacagccttctggaagagaccaagcaaggtaatctggagagagagtgtatcgaggaactttgtaacaaagaggaagcacgcgaagtatttgaaaatgacccggaaaccgattatttttacccaaaatatctcgta

SEQ ID NO: 16 - protein, 12 aa, Artificial Sequence
  modified IgG4 hinge
ESKYGPPCPPCP

SEQ ID NO: 17 - protein, 13 aa, Homo sapiens
  TLR4 juxtamembrane domain
PVLSLNITCQMNK

SEQ ID NO: 18 - protein, 21 aa, Homo sapiens
  Tim1 transmembrane domain
IYAGVCISVLVLLALLGVIIA

SEQ ID NO: 19 - protein, 21 aa, Homo sapiens
  Tim4 transmembrane domain
LLMIIAPSLGFVLFALFVAFL

SEQ ID NO: 20 - protein, 21 aa, Homo sapiens
  FcgammaRI transmembrane domain
VLFYLAVGIMFLVNTVLWVTI

SEQ ID NO: 21 - protein, 21 aa, Homo sapiens
  FcepsilonRIgamma transmembrane domain
LCYILDAILFLYGIVLTLLYC

SEQ ID NO: 22 - protein, 21 aa, Homo sapiens
  CD8a transmembrane domain
IYIWAPLAGTCGVLLLSLVIT

SEQ ID NO: 23 - protein, 21 aa, Homo sapiens
  MERTK transmembrane domain
FGCFCGFILIGLILYISLAIR

SEQ ID NO: 24 - protein, 21 aa, Homo sapiens
  Axl transmembrane domain
YVLLGAVVAAACVLILALFLV

SEQ ID NO: 25 - protein, 21 aa, Homo sapiens
  Tyro3 transmembrane domain
VPVVLGVLTALVTAAALALIL

SEQ ID NO: 26 - protein, 27 aa, Homo sapiens
  CD28 transmembrane domain
FWVLVVVGGVLACYSLLVTVAFIIFWV

SEQ ID NO: 27 - protein, 22 aa, Homo sapiens
  CD4 transmembrane domain
MALIVLGGVAGLLLFIGLGIFF

SEQ ID NO: 28 - protein, 21 aa, Homo sapiens
  DAP12 transmembrane domain
GVLAGIVMGDLVLTVLIALAV

SEQ ID NO: 29 - protein, 21 aa, Homo sapiens
  BAI1 transmembrane domain
VTLIVGCGVSSLTLLMLVIIY

SEQ ID NO: 30 - protein, 21 aa, Homo sapiens
  MRC1 transmembrane domain
GVVIIVILLILTGAGLAAYFF

SEQ ID NO: 31 - protein, 21 aa, Homo sapiens
  TLR1 transmembrane domain
LLIVTIVATMLVLAVTVTSLC

SEQ ID NO: 32 - protein, 21 aa, Homo sapiens
  TLR2 transmembrane domain
ALVSGMCCALFLLILLTGVLC

SEQ ID NO: 33 - protein, 21 aa, Homo sapiens
  TLR3 Transmembrane domain
FFMINTSILLIFIFIVLLIHF

SEQ ID NO: 34 - protein, 21 aa, Homo sapiens
  TLR4 transmembrane domain
TIIGVSVLSVLVVSVVAVLVY

SEQ ID NO: 35 - protein, 21 aa, Homo sapiens
  TLR5 transmembrane domain
FSLFIVCTVTLTLFLMTILTV

SEQ ID NO: 36 - protein, 21 aa, Homo sapiens
  TLR6 transmembrane domain
ALVSGMCCALFLLILLTGVLC

SEQ ID NO: 37 - protein, 21 aa, Homo sapiens
  TLR7 transmembrane domain
LILFSLSISVSLFLMVMMTAS

SEQ ID NO: 38 - protein, 21 aa, Homo sapiens
  TLR8 transmembrane domain
AVILFFFTFFITTMVMLAALA

SEQ ID NO: 39 - protein, 21 aa, Homo sapiens
  TLR9 transmembrane domain
FALSLLAVALGLGVPMLHHLC

SEQ ID NO: 40 - DNA, 63 bp, Homo sapiens
  misc_feature: Tim1 transmembrane domain
atatacgctggagtctgtataagtgtccttgtactgttggcgttgctgggggtcattattgcc

SEQ ID NO: 41 - DNA, 63 bp, Homo sapiens
  misc_feature: Tim4 transmembrane domain
ttgcttatgattattgcgccaagccttggatttgtgctgttcgcactcttcgtagcttttctc

SEQ ID NO: 42 - DNA, 63 bp, Homo sapiens
  misc_feature: FcgammaRI transmembrane domain
gtactgttttatctcgccgtagggataatgttcctcgtgaacaccgtactgtgggtaacaata

SEQ ID NO: 43 - DNA, 63 bp, Homo sapiens
  misc_feature: CD8a transmembrane domain
atatacatttgggcaccgctggctggaacttgcggcgttctcttgttgagtctggtgattact

SEQ ID NO: 44 - DNA, 63 bp, Homo sapiens
  misc_feature: MERTK transmembrane domain
tttggctgtttctgtggatttattctgattggtcttatcctctatatttccttggcgatcaga

SEQ ID NO: 45 - DNA, 63 bp, Homo sapiens
  misc_feature: Axl transmembrane domain
tatgtcttgcttggtgccgtcgttgctgccgcctgtgtgttgatactcgcacttttcttggtg

SEQ ID NO: 46 - DNA, 63 bp, Homo sapiens
  misc_feature: Tyro3 transmembrane domain
gtacccgtcgttttgggggtcctgaccgcgctcgttactgcggcagcactcgcactgatactt

SEQ ID NO: 47 - DNA, 66 bp, Homo sapiens
  misc_feature: CD4 transmembrane domain
atggctctgatcgtactgggcggagtggcaggattgctgctctttattggactgggcattttcttc

SEQ ID NO: 48 - protein, 185 aa, Homo sapiens
  TLR1 signaling domain
SYLDLPWYLRMVCQWTQTRRRARNIPLEELQRNLQFHAFISYSGHDSFWVKNELLPNLEKEGMQICLHERNFVPGKSIVENIITCIEKSYKSIFVLSPNFVQSEWCHYELYFAHHNLFHEGSNSLILILLEPIPQYSIPSSYHKLKSLMARRTYLEWPKEKSKRGLFWANLRAAINIKLTEQAKK

SEQ ID NO: 49 - protein, 175 aa, Homo sapiens
  TLR2 signaling domain
HRFHGLWYMKMMWAWLQAKRKPRKAPSRNICYDAFVSYSERDAYWVENLMVQELENFNPPFKLCLHKRDFIPGKWIIDNIIDSIEKSHKTVFVLSENFVKSEWCKYELDFSHFRLFDENNDAAILILLEPIEKKAIPQRFCKLRKIMNTKTYLEWPMDEAQREGFWVNLRAAIKS

SEQ ID NO: 50 - protein, 179 aa, Homo sapiens
  TLR3 signaling domain
EGWRISFYWNVSVHRVLGFKEIDRQTEQFEYAAYIIHAYKDKDWVWEHFSSMEKEDQSLKFCLEERDFEAGVFELEAIVNSIKRSRKIIFVITHHLLKDPLCKRFKVHHAVQQAIEQNLDSIILVFLEEIPDYKLNHALCLRRGMFKSHCILNWPVQKERIGAFRHKLQVALGSKNSVH

SEQ ID NO: 51 - protein, 187 aa, Homo sapiens
  TLR4 signaling domain
KFYFHLMLLAGCIKYGRGENIYDAFVIYSSQDEDWVRNELVKNLEEGVPPFQLCLHYRDFIPGVAIAANIIHEGFHKSRKVIVVVSQHFIQSRWCIFEYEIAQTWQFLSSRAGIIFIVLQKVEKTLLRQQVELYRLLSRNTYLEWEDSVLGRHIFWRRLRKALLDGKSWNPEGTVGTGCNWQEATSI

SEQ ID NO: 52 - protein, 198 aa, Homo sapiens
  TLR5 signaling domain
TKFRGFCFICYKTAQRLVFKDHPQGTEPDMYKYDAYLCFSSKDFTWVQNALLKHLDTQYSDQNRFNLCFEERDFVPGENRIANIQDAIWNSRKIVCLVSRHFLRDGWCLEAFSYAQGRCLSDLNSALIMVVVGSLSQYQLMKHQSIRGFVQKQQYLRWPEDFQDVGWFLHKLSQQILKKEKEKKKDNNIPLQTVATIS

SEQ ID NO: 53 - protein, 189 aa, Homo sapiens
  TLR6 signaling domain
YLDLPWYLRMVCQWTQTRRRARNIPLEELQRNLQFHAFISYSEHDSAWVKSELVPYLEKEDIQICLHERNFVPGKSIVENIINCIEKSYKSIFVLSPNFVQSEWCHYELYFAHHNLFHEGSNNLILILLEPIPQNSIPNKYHKLKALMTQRTYLQWPKEKSKRGLFWANIRAAFNMKLTLVTENNDVKS

SEQ ID NO: 54 - protein, 189 aa, Homo sapiens
  TLR7 signaling domain
HLYFWDVWYIYHFCKAKIKGYQRLISPDCCYDAFIVYDTKDPAVTEWVLAELVAKLEDPREKHFNLCLEERDWLPGQPVLENLSQSIQLSKKTVFVMTDKYAKTENFKIAFYLSHQRLMDEKVDVIILIFLEKPFQKSKFLQLRKRLCGSSVLEWPTNPQAHPYFWQCLKNALATDNHVAYSQVFKETV

SEQ ID NO: 55 - protein, 193 aa, Homo sapiens
  TLR8 signaling domain
HHLFYWDVWFIYNVCLAKVKGYRSLSTSQTFYDAYISYDTKDASVTDWVINELRYHLEESRDKNVLLCLEERDWDPGLAIIDNLMQSINQSKKTVFVLTKKYAKSWNFKTAFYLALQRLMDENMDVIIFILLEPVLQHSQYLRLRQRICKSSILQWPDNPKAEGLFWQTLRNVVLTENDSRYNNMYVDSIKQY

SEQ ID NO: 56 - protein, 193 aa, Homo sapiens
  TLR9 signaling domain
GWDLWYCFHLCLAWLPWRGRQSGRDEDALPYDAFVVFDKTQSAVADWVYNELRGQLEECRGRWALRLCLEERDWLPGKTLFENLWASVYGSRKTLFVLAHTDRVSGLLRASFLLAQQRLLEDRKDVVVLVILSPDGRRSRYVRLRQRLCRQSVLLWPHQPSGQRSFWAQLGMALTRDNHHFYNRNFCQGPTAE

SEQ ID NO: 57 - protein, 522 aa, Homo sapiens
  Traf6 signaling domain - full length
MSLLNCENSCGSSQSESDCCVAMASSCSAVTKDDSVGGTASTGNLSSSFMEEIQGYDVEFDPPLESKYECPICLMALREAVQTPCGHRFCKACIIKSIRDAGHKCPVDNEILLENQLFPDNFAKREILSLMVKCPNEGCLHKMELRHLEDHQAHCEFALMDCPQCQRPFQKFHINIHILKDCPRRQVSCDNCAASMAFEDKEIHDQNCPLANVICEYCNTILIREQMPNHYDLDCPTAPIPCTFSTFGCHEKMQRNHLARHLQENTQSHMRMLAQAVHSLSVIPDSGYISEVRNFQETIHQLEGRLVRQDHQIRELTAKMETQSMYVSELKRTIRTLEDKVAEIEAQQCNGIYIWKIGNFGMHLKCQEEEKPVVIHSPGFYTGKPGYKLCMRLHLQLPTAQRCANYISLFVHTMQGEYDSHLPWPFQGTIRLTILDQSEAPVRQNHEEIMDAKPELLAFQRPTIPRNPKGFGYVTFMHLEALRQRTFIKDDTLLVRCEVSTRFDMGSLRREGFQPRSTDAGV

SEQ ID NO: 58 - protein, 274 aa, Homo sapiens
  truncated TRAF6 signaling domain
MSLLNCENSCGSSQSESDCCVAMASSCSAVTKDDSVGGTASTGNLSSSFMEEIQGYDVEFDPPLESKYECPICLMALREAVQTPCGHRFCKACIIKSIRDAGHKCPVDNEILLENQLFPDNFAKREILSLMVKCPNEGCLHKMELRHLEDHQAHCEFALMDCPQCQRPFQKFHINIHILKDCPRRQVSCDNCAASMAFEDKEIHDQNCPLANVICEYCNTILIREQMPNHYDLDCPTAPIPCTFSTFGCHEKMQRNHLARHLQENTQSHMRMLA

SEQ ID NO: 59 - protein, 473 aa, Homo sapiens
  MERTK signaling domain
KRVQETKFGNAFTEEDSELVVNYIAKKSFCRRAIELTLHSLGVSEELQNKLEDVVIDRNLLILGKILGEGEFGSVMEGNLKQEDGTSLKVAVKTMKLDNSSQREIEEFLSEAACMKDFSHPNVIRLLGVCIEMSSQGIPKPMVILPFMKYGDLHTYLLYSRLETGPKHIPLQTLLKFMVDIALGMEYLSNRNFLHRDLAARNCMLRDDMTVCVADFGLSKKIYSGDYYRQGRIAKMPVKWIAIESLADRVYTSKSDVWAFGVTMWEIATRGMTPYPGVQNHEMYDYLLHGHRLKQPEDCLDELYEIMYSCWRTDPLDRPTFSVLRLQLEKLLESLPDVRNQADVIYVNTQLLESSEGLAQGSTLAPLDLNIDPDSIIASCTPRAAISVVTAEVHDSKPHEGRYILNGGSEEWEDLTSAPSAAVTAEKNSVLPGERLVRNGVSWSHSSMLPLGSSLPDELLFADDSSEGSEVLM

SEQ ID NO: 60-61 - skipped (2 entries)

SEQ ID NO: 62 - protein, 42 aa, Homo sapiens
  FcepsilonRIgamma signaling domain
RLKIQVRKAAITSYEKSDGVYTGLSTRNQETYETLKHEKPPQ

SEQ ID NO: 63 - protein, 61 aa, Homo sapiens
  FcgammaR1 signaling domain
RKELKRKKKWDLEISLDSGHEKKVISSLQEDRHLEEELKCQEQKEEQLQEGVHRKEPQGAT

SEQ ID NO: 64 - protein, 77 aa, Homo sapiens
  FcgammaR2A signaling domain
CRKKRISANSTDPVKAAQFEPPGRQMIAIRKRQLEETNNDYETADGGYMTLNPRAPTDDDKNIYLTLPPNDHVNSNN

SEQ ID NO: 65 - protein, 77 aa, Homo sapiens
  FcgammaR2c signaling domain
CRKKRISANSTDPVKAAQFEPPGRQMIAIRKRQPEETNNDYETADGGYMTLNPRAPTDDDKNIYLTLPPNDHVNSNN

SEQ ID NO: 66 - protein, 25 aa, Homo sapiens
  FcgammaR3A signaling domain
KTNIRSSTRDWKDHKFKWRKDPQDK

SEQ ID NO: 67 - protein, 85 aa, Homo sapiens
  BAFF-R signaling domain
SWRRRQRRLRGASSAEAPDGDKDAPEPLDKVIILSPGISDATAPAWPPPGEDPGTTPPGHSVPVPATELGSTELVTTKTAGPEQQ

SEQ ID NO: 68 - protein, 52 aa, Homo sapiens
  DAP12 signaling domain
YFLGRLVPRGRGAAEAATRKQRITETESPYQELQGQRSDVYSDLNTQRPYYK

SEQ ID NO: 69 - protein, 86 aa, Homo sapiens
  NFAM1 signaling domain
LWNKKRMRGPGKDPTRKCPDPRSASSPKQHPSESVYTALQRRETEVYACIENEDGSSPTAKQSPLSQERPHRFEDDGELNLVYENL

SEQ ID NO: 70 - protein, 29 aa, Homo sapiens
  truncated NFAM1 signaling domain
SSPKQHPSESVYTALQRRETEVYACIENE

SEQ ID NO: 71 - protein, 29 aa, Homo sapiens
  CD79b truncated signaling domain (185-213)
DSKAGMEEDHTYEGLDIDQTATYEDIVTL

SEQ ID NO: 72 - protein, 303 aa, Homo sapiens
  TRAF2 signaling domain
MAAASVTPPGSLELLQPGFSKTLLGTKLEAKYLCSACRNVLRRPFQAQCGHRYCSFCLASILSSGPQNCAACVHEGIYEEGISILESSSAFPDNAARREVESLPAVCPSDGCTWKGTLKEYESCHEGRCPLMLTECPACKGLVRLGEKERHLEHECPERSLSCRHCRAPCCGADVKAHHEVCPKFPLTCDGCGKKKIPREKFQDHVKTCGKCRVPCRFHAIGCLETVEGEKQQEHEVQWLREHLAMLLSSVLEAKPLLGDQSHAGSELLQRCESLEKKTATFENIVCVLNREVERVAMTAEAC

SEQ ID NO: 73 - protein, 274 aa, Homo sapiens
  TRAF3 signaling domain
MESSKKMDSPGALQTNPPLKLHTDRSAGTPVFVPEQGGYKEKFVKTVEDKYKCEKCHLVLCSPKQTECGHRFCESCMAALLSSSSPKCTACQESIVKDKVFKDNCCKREILALQIYCRNESRGCAEQLMLGHLLVHLKNDCHFEELPCVRPDCKEKVLRKDLRDHVEKACKYREATCSHCKSQVPMIALQKHEDTDCPCVVVSCPHKCSVQTLLRSELSAHLSECVNAPSTCSFKRYGCVFQGTNQQIKAHEASSAVQHVNLLKEWSNSLEKKV

SEQ ID NO: 74 - DNA, 1566 bp, Homo sapiens
  misc_feature: Traf6 signaling domain - full length
atgtcactccttaactgcgaaaacagttgtgggagttcacaatccgaaagtgattgttgcgtggcgatggcgtcttcatgctctgcggttaccaaggatgactctgtgggaggcaccgcatctaccggaaatctgagctcttcttttatggaggaaattcagggctacgacgttgagtttgatcctcctctcgaatctaagtatgagtgccccatatgtctcatggcgttgagagaagcagtgcagactccgtgcggacatcgcttctgcaaggcgtgtattataaagagtatacgcgatgcgggtcacaaatgtccagtggacaacgagatactgcttgaaaatcaacttttccccgacaattttgcaaagagagagatactgtctttgatggttaagtgtccaaacgagggctgcttgcacaaaatggaactccgacaccttgaagaccaccaggcacactgcgagttcgccctcatggattgcccacaatgccagcgcccgttccaaaagtttcacataaacatccacatactgaaggactgtcctaggagacaagtaagctgtgacaattgcgcagcgtcaatggcgttcgaggacaaggagatacacgatcaaaactgtcctctggcgaatgtgatctgcgaatattgcaatacgatcttgatccgcgaacagatgcctaatcattacgacctcgattgtccgaccgcgccaattccttgtactttttctaccttcggatgtcatgagaaaatgcaacgaaatcacctggctcgccatcttcaggagaatactcagagccacatgcgcatgttggctcaagccgtacatagccttagcgtaataccggactcaggttatatatccgaagtacggaattttcaagaaaccatacatcaacttgaaggaaggttggtacgacaggatcatcagatacgcgaattgacggccaagatggaaacccagagcatgtatgtcagtgagcttaagcgcactatccgaaccctggaggataaagttgccgaaatcgaagctcaacaatgcaacgggatatacatttggaaaataggtaacttcggaatgcacctgaagtgtcaagaagaagaaaaacctgtcgttattcattcccccggcttttatacagggaagcctgggtataagctttgcatgaggctccacctccaattgccgacggcgcaaaggtgcgcaaattacatttctctgtttgtccatactatgcagggtgagtacgatagtcacttgccgtggcccttccagggtaccatacgattgaccatcctggatcagagcgaggcccccgtgcgacagaatcatgaagaaataatggatgctaagccggaactgctcgctttccagagacctacaattccgcgaaatcctaagggttttggctatgttacgttcatgcatctggaagcactcagacaaagaacattcattaaagatgacaccttgcttgtgcggtgtgaggtgtcaaccaggttcgacatgggatctctcagacgggaggggttccaaccgcgctctacagacgctggagtg

SEQ ID NO: 75 - protein, 45 aa, Homo sapiens
  CD79b signaling domain (185-229)
DSKAGMEEDHTYEGLDIDQTATYEDIVTLRTGEVKWSVGEHPGQE

SEQ ID NO: 76 - protein, 141 aa, Homo sapiens
  MyD88 TIR domain
HMPERFDAFICYCPSDIQFVQEMIRQLEQTNYRLKLCVSDRDVLPGTCVWSIASELIEKRCRRMVVVVSDDYLQSKECDFQTKFALSLSPGAHQKRLIPIKYKAMKKEFPSILRFITVCDYTNPCTKSWFWTRLAKALSLP

SEQ ID NO: 77 - DNA, 183 bp, Homo sapiens
  misc_feature: FcgammaR1 signaling domain
agaaaggaactcaagcgcaagaagaagtgggacctggagatttctctcgactccggtcacgaaaagaaggtcatcagtagcttgcaagaggaccgacacttggaagaagaacttaaatgccaggaacagaaagaggagcagctccaggagggagtccaccggaaagaaccacagggagcaact

SEQ ID NO: 78 - DNA, 231 bp, Homo sapiens
  misc_feature: FcgammaR2A signaling domain
tgtcgaaagaagcggatttcagccaatagtacagacccagtgaaagccgctcaatttgagccacccggtcgacagatgatcgcaattaggaaacgccaactggaggaaacgaataatgattacgaaacggcagatgggggctacatgacgctcaatcctagagctccgaccgacgacgacaagaatatatatctgactctccctcccaacgaccacgtaaacagtaataac

SEQ ID NO: 79 - DNA, 231 bp, Homo sapiens
  misc_feature: FcgammaR2C signaling domain
tgcagaaagaagcggataagtgcaaatagtactgatcccgttaaagcagcacaatttgagccgccaggacggcaaatgattgcaatcagaaaacgacaacccgaggaaaccaataatgactacgagaccgctgacggagggtatatgacgttgaatccccgcgcaccaacggatgacgataagaacatttatcttacgctgccccctaacgatcatgtgaatagcaataac

SEQ ID NO: 80 - DNA, 75 bp, Homo sapiens
  misc_feature: FcgammaR3A signaling domain
aaaacaaatatccggtcctctacgagggactggaaagatcataaattcaagtggagaaaagatcctcaggataaa

SEQ ID NO: 81 - protein, 487 aa, Artificial Sequence
  CER05 chimeric engulfment receptor
  sig_peptide 1...22
MSKGLLLLWLVTELWWLYLTPAASEDTIIGFLGQPVTLPCHYLSWSQSRNSMCWGKGSCPNSKCNAELLRTDGTRIISRKSTKYTLLGKVQFGEVSLTISNTNRGDSGVYCCRIEVPGWFNDVKKNVRLELRRATTTKKPTTTTRPTTTPYVTTTTPELLPTTVMTTSVLPTTTPPQTLATTAFSTAVTTCPSTTPGSFSQETTKGSAFTTESETLPASNHSQRSMMTISTDIAVLRPTGSNPGILPSTSQLTTQKTTLTTSESLQKTTKSHQINSRQTILIIACCVGFVLMVLLFLAFLKFYFHLMLLAGCIKYGRGENIYDAFVIYSSQDEDWVRNELVKNLEEGVPPFQLCLHYRDFIPGVAIAANIIHEGFHKSRKVIVVVSQHFIQSRWCIFEYEIAQTWQFLSSRAGIIFIVLQKVEKTLLRQQVELYRLLSRNTYLEWEDSVLGRHIFWRRLRKALLDGKSWNPEGTVGTGCNWQEATSI

SEQ ID NO: 82 - protein, 487 aa, Artificial Sequence
  CER06 chimeric engulfment receptor
  sig_peptide 1...22
MSKGLLLLWLVTELWWLYLTPAASEDTIIGFLGQPVTLPCHYLSWSQSRNSMCWGKGSCPNSKCNAELLRTDGTRIISRKSTKYTLLGKVQFGEVSLTISNTNRGDSGVYCCRIEVPGWFNDVKKNVRLELRRATTTKKPTTTTRPTTTPYVTTTTPELLPTTVMTTSVLPTTTPPQTLATTAFSTAVTTCPSTTPGSFSQETTKGSAFTTESETLPASNHSQRSMMTISTDIAVLRPTGSNPGILPSTSQLTTQKTTLTTSESLQKTTKSHQINSRQTTIIGVSVLSVLVVSVVAVLVYKFYFHLMLLAGCIKYGRGENIYDAFVIYSSQDEDWVRNELVKNLEEGVPPFQLCLHYRDFIPGVAIAANIIHEGFHKSRKVIVVVSQHFIQSRWCIFEYEIAQTWQFLSSRAGIIFIVLQKVEKTLLRQQVELYRLLSRNTYLEWEDSVLGRHIFWRRLRKALLDGKSWNPEGTVGTGCNWQEATSI

SEQ ID NO: 83 - protein, 500 aa, Artificial Sequence
  CER07 chimeric engulfment receptor
  sig_peptide 1...22
MSKGLLLLWLVTELWWLYLTPAASEDTIIGFLGQPVTLPCHYLSWSQSRNSMCWGKGSCPNSKCNAELLRTDGTRIISRKSTKYTLLGKVQFGEVSLTISNTNRGDSGVYCCRIEVPGWFNDVKKNVRLELRRATTTKKPTTTTRPTTTPYVTTTTPELLPTTVMTTSVLPTTTPPQTLATTAFSTAVTTCPSTTPGSFSQETTKGSAFTTESETLPASNHSQRSMMTISTDIAVLRPTGSNPGILPSTSQLTTQKTTLTTSESLQKTTKSHQINSRQTPVLSLNITCQMNKTIIGVSVLSVLVVSVVAVLVYKFYFHLMLLAGCIKYGRGENIYDAFVIYSSQDEDWVRNELVKNLEEGVPPFQLCLHYRDFIPGVAIAANIIHEGFHKSRKVIVVVSQHFIQSRWCIFEYEIAQTWQFLSSRAGIIFIVLQKVEKTLLRQQVELYRLLSRNTYLEWEDSVLGRHIFWRRLRKALLDGKSWNPEGTVGTGCNWQEATSI

SEQ ID NO: 84 - protein, 479 aa, Artificial Sequence
  CER17 chimeric engulfment receptor
  sig_peptide 1...22
MSKGLLLLWLVTELWWLYLTPAASEDTIIGFLGQPVTLPCHYLSWSQSRNSMCWGKGSCPNSKCNAELLRTDGTRIISRKSTKYTLLGKVQFGEVSLTISNTNRGDSGVYCCRIEVPGWFNDVKKNVRLELRRATTTKKPTTTTRPTTTPYVTTTTPELLPTTVMTTSVLPTTTPPQTLATTAFSTAVTTCPSTTPGSFSQETTKGSAFTTESETLPASNHSQRSMMTISTDIAVLRPTGSNPGILPSTSQLTTQKTTLTTSESLQKTTKSHQINSRQTILIIACCVGFVLMVLLFLAFLEGWRISFYWNVSVHRVLGFKEIDRQTEQFEYAAYIIHAYKDKDWVWEHFSSMEKEDQSLKFCLEERDFEAGVFELEAIVNSIKRSRKIIFVITHHLLKDPLCKRFKVHHAVQQAIEQNLDSIILVFLEEIPDYKLNHALCLRRGMFKSHCILNWPVQKERIGAFRHKLQVALGSKNSVH

SEQ ID NO: 85 - protein, 479 aa, Artificial Sequence
  CER18 chimeric engulfment receptor
  sig_peptide 1...22
MSKGLLLLWLVTELWWLYLTPAASEDTIIGFLGQPVTLPCHYLSWSQSRNSMCWGKGSCPNSKCNAELLRTDGTRIISRKSTKYTLLGKVQFGEVSLTISNTNRGDSGVYCCRIEVPGWFNDVKKNVRLELRRATTTKKPTTTTRPTTTPYVTTTTPELLPTTVMTTSVLPTTTPPQTLATTAFSTAVTTCPSTTPGSFSQETTKGSAFTTESETLPASNHSQRSMMTISTDIAVLRPTGSNPGILPSTSQLTTQKTTLTTSESLQKTTKSHQINSRQTFFMINTSILLIFIFIVLLIHFEGWRISFYWNVSVHRVLGFKEIDRQTEQFEYAAYIIHAYKDKDWVWEHFSSMEKEDQSLKFCLEERDFEAGVFELEAIVNSIKRSRKIIFVITHHLLKDPLCKRFKVHHAVQQAIEQNLDSIILVFLEEIPDYKLNHALCLRRGMFKSHCILNWPVQKERIGAFRHKLQVALGSKNSVH

SEQ ID NO: 86 - protein, 498 aa, Artificial Sequence
  CER19 chimeric engulfment receptor
  sig_peptide 1...22
MSKGLLLLWLVTELWWLYLTPAASEDTIIGFLGQPVTLPCHYLSWSQSRNSMCWGKGSCPNSKCNAELLRTDGTRIISRKSTKYTLLGKVQFGEVSLTISNTNRGDSGVYCCRIEVPGWFNDVKKNVRLELRRATTTKKPTTTTRPTTTPYVTTTTPELLPTTVMTTSVLPTTTPPQTLATTAFSTAVTTCPSTTPGSFSQETTKGSAFTTESETLPASNHSQRSMMTISTDIAVLRPTGSNPGILPSTSQLTTQKTTLTTSESLQKTTKSHQINSRQTILIIACCVGFVLMVLLFLAFLTKFRGFCFICYKTAQRLVFKDHPQGTEPDMYKYDAYLCFSSKDFTWVQNALLKHLDTQYSDQNRFNLCFEERDFVPGENRIANIQDAIWNSRKIVCLVSRHFLRDGWCLEAFSYAQGRCLSDLNSALIMVVVGSLSQYQLMKHQSIRGFVQKQQYLRWPEDFQDVGWFLHKLSQQILKKEKEKKKDNNIPLQTVATIS

SEQ ID NO: 87 - protein, 498 aa, Artificial Sequence
  CER20 chimeric engulfment receptor
  sig_peptide 1...22
MSKGLLLLWLVTELWWLYLTPAASEDTIIGFLGQPVTLPCHYLSWSQSRNSMCWGKGSCPNSKCNAELLRTDGTRIISRKSTKYTLLGKVQFGEVSLTISNTNRGDSGVYCCRIEVPGWFNDVKKNVRLELRRATTTKKPTTTTRPTTTPYVTTTTPELLPTTVMTTSVLPTTTPPQTLATTAFSTAVTTCPSTTPGSFSQETTKGSAFTTESETLPASNHSQRSMMTISTDIAVLRPTGSNPGILPSTSQLTTQKTTLTTSESLQKTTKSHQINSRQTFSLFIVCTVTLTLFLMTILTVTKFRGFCFICYKTAQRLVFKDHPQGTEPDMYKYDAYLCFSSKDFTWVQNALLKHLDTQYSDQNRFNLCFEERDFVPGENRIANIQDAIWNSRKIVCLVSRHFLRDGWCLEAFSYAQGRCLSDLNSALIMVVVGSLSQYQLMKHQSIRGFVQKQQYLRWPEDFQDVGWFLHKLSQQILKKEKEKKKDNNIPLQTVATIS

SEQ ID NO: 88 - protein, 493 aa, Artificial Sequence
  CER21 chimeric engulfment receptor
  sig_peptide 1...22
MSKGLLLLWLVTELWWLYLTPAASEDTIIGFLGQPVTLPCHYLSWSQSRNSMCWGKGSCPNSKCNAELLRTDGTRIISRKSTKYTLLGKVQFGEVSLTISNTNRGDSGVYCCRIEVPGWFNDVKKNVRLELRRATTTKKPTTTTRPTTTPYVTTTTPELLPTTVMTTSVLPTTTPPQTLATTAFSTAVTTCPSTTPGSFSQETTKGSAFTTESETLPASNHSQRSMMTISTDIAVLRPTGSNPGILPSTSQLTTQKTTLTTSESLQKTTKSHQINSRQTILIIACCVGFVLMVLLFLAFLHHLFYWDVWFIYNVCLAKVKGYRSLSTSQTFYDAYISYDTKDASVTDWVINELRYHLEESRDKNVLLCLEERDWDPGLAIIDNLMQSINQSKKTVFVLTKKYAKSWNFKTAFYLALQRLMDENMDVIIFILLEPVLQHSQYLRLRQRICKSSILQWPDNPKAEGLFWQTLRNVVLTENDSRYNNMYVDSIKQY

SEQ ID NO: 89 - protein, 493 aa, Artificial Sequence
  CER22 chimeric engulfment receptor
  sig_peptide 1...22
MSKGLLLLWLVTELWWLYLTPAASEDTIIGFLGQPVTLPCHYLSWSQSRNSMCWGKGSCPNSKCNAELLRTDGTRIISRKSTKYTLLGKVQFGEVSLTISNTNRGDSGVYCCRIEVPGWFNDVKKNVRLELRRATTTKKPTTTTRPTTTPYVTTTTPELLPTTVMTTSVLPTTTPPQTLATTAFSTAVTTCPSTTPGSFSQETTKGSAFTTESETLPASNHSQRSMMTISTDIAVLRPTGSNPGILPSTSQLTTQKTTLTTSESLQKTTKSHQINSRQTAVILFFFTFFITTMVMLAALAHHLFYWDVWFIYNVCLAKVKGYRSLSTSQTFYDAYISYDTKDASVTDWVINELRYHLEESRDKNVLLCLEERDWDPGLAIIDNLMQSINQSKKTVFVLTKKYAKSWNFKTAFYLALQRLMDENMDVIIFILLEPVLQHSQYLRLRQRICKSSILQWPDNPKAEGLFWQTLRNVVLTENDSRYNNMYVDSIKQY

SEQ ID NO: 90 - protein, 493 aa, Artificial Sequence
  CER23 chimeric engulfment receptor
  sig_peptide 1...22
MSKGLLLLWLVTELWWLYLTPAASEDTIIGFLGQPVTLPCHYLSWSQSRNSMCWGKGSCPNSKCNAELLRTDGTRIISRKSTKYTLLGKVQFGEVSLTISNTNRGDSGVYCCRIEVPGWFNDVKKNVRLELRRATTTKKPTTTTRPTTTPYVTTTTPELLPTTVMTTSVLPTTTPPQTLATTAFSTAVTTCPSTTPGSFSQETTKGSAFTTESETLPASNHSQRSMMTISTDIAVLRPTGSNPGILPSTSQLTTQKTTLTTSESLQKTTKSHQINSRQTILIIACCVGFVLMVLLFLAFLGWDLWYCFHLCLAWLPWRGRQSGRDEDALPYDAFVVFDKTQSAVADWVYNELRGQLEECRGRWALRLCLEERDWLPGKTLFENLWASVYGSRKTLFVLAHTDRVSGLLRASFLLAQQRLLEDRKDVVVLVILSPDGRRSRYVRLRQRLCRQSVLLWPHQPSGQRSFWAQLGMALTRDNHHFYNRNFCQGPTAE

SEQ ID NO: 91 - protein, 493 aa, Artificial Sequence
  CER24 chimeric engulfment receptor
  sig_peptide 1...22
MSKGLLLLWLVTELWWLYLTPAASEDTIIGFLGQPVTLPCHYLSWSQSRNSMCWGKGSCPNSKCNAELLRTDGTRIISRKSTKYTLLGKVQFGEVSLTISNTNRGDSGVYCCRIEVPGWFNDVKKNVRLELRRATTTKKPTTTTRPTTTPYVTTTTPELLPTTVMTTSVLPTTTPPQTLATTAFSTAVTTCPSTTPGSFSQETTKGSAFTTESETLPASNHSQRSMMTISTDIAVLRPTGSNPGILPSTSQLTTQKTTLTTSESLQKTTKSHQINSRQTFALSLLAVALGLGVPMLHHLCGWDLWYCFHLCLAWLPWRGRQSGRDEDALPYDAFVVFDKTQSAVADWVYNELRGQLEECRGRWALRLCLEERDWLPGKTLFENLWASVYGSRKTLFVLAHTDRVSGLLRASFLLAQQRLLEDRKDVVVLVILSPDGRRSRYVRLRQRLCRQSVLLWPHQPSGQRSFWAQLGMALTRDNHHFYNRNFCQGPTAE

SEQ ID NO: 92 - protein, 485 aa, Artificial Sequence
  CER26 chimeric engulfment receptor
  sig_peptide 1...22
MSKGLLLLWLVTELWWLYLTPAASEDTIIGFLGQPVTLPCHYLSWSQSRNSMCWGKGSCPNSKCNAELLRTDGTRIISRKSTKYTLLGKVQFGEVSLTISNTNRGDSGVYCCRIEVPGWFNDVKKNVRLELRRATTTKKPTTTTRPTTTPYVTTTTPELLPTTVMTTSVLPTTTPPQTLATTAFSTAVTTCPSTTPGSFSQETTKGSAFTTESETLPASNHSQRSMMTISTDIAVLRPTGSNPGILPSTSQLTTQKTTLTTSESLQKTTKSHQINSRQTILIIACCVGFVLMVLLFLAFLSYLDLPWYLRMVCQWTQTRRRARNIPLEELQRNLQFHAFISYSGHDSFWVKNELLPNLEKEGMQICLHERNFVPGKSIVENIITCIEKSYKSIFVLSPNFVQSEWCHYELYFAHHNLFHEGSNSLILILLEPIPQYSIPSSYHKLKSLMARRTYLEWPKEKSKRGLFWANLRAAINIKLTEQAKK

SEQ ID NO: 93 - protein, 475 aa, Artificial Sequence
  CER27 chimeric engulfment receptor
  sig_peptide 1...22
MSKGLLLLWLVTELWWLYLTPAASEDTIIGFLGQPVTLPCHYLSWSQSRNSMCWGKGSCPNSKCNAELLRTDGTRIISRKSTKYTLLGKVQFGEVSLTISNTNRGDSGVYCCRIEVPGWFNDVKKNVRLELRRATTTKKPTTTTRPTTTPYVTTTTPELLPTTVMTTSVLPTTTPPQTLATTAFSTAVTTCPSTTPGSFSQETTKGSAFTTESETLPASNHSQRSMMTISTDIAVLRPTGSNPGILPSTSQLTTQKTTLTTSESLQKTTKSHQINSRQTILIIACCVGFVLMVLLFLAFLHRFHGLWYMKMMWAWLQAKRKPRKAPSRNICYDAFVSYSERDAYWVENLMVQELENFNPPFKLCLHKRDFIPGKWIIDNIIDSIEKSHKTVFVLSENFVKSEWCKYELDFSHFRLFDENNDAAILILLEPIEKKAIPQRFCKLRKIMNTKTYLEWPMDEAQREGFWVNLRAAIKS

SEQ ID NO: 94 - protein, 489 aa, Artificial Sequence
  CER28 chimeric engulfment receptor
  sig_peptide 1...22
MSKGLLLLWLVTELWWLYLTPAASEDTIIGFLGQPVTLPCHYLSWSQSRNSMCWGKGSCPNSKCNAELLRTDGTRIISRKSTKYTLLGKVQFGEVSLTISNTNRGDSGVYCCRIEVPGWFNDVKKNVRLELRRATTTKKPTTTTRPTTTPYVTTTTPELLPTTVMTTSVLPTTTPPQTLATTAFSTAVTTCPSTTPGSFSQETTKGSAFTTESETLPASNHSQRSMMTISTDIAVLRPTGSNPGILPSTSQLTTQKTTLTTSESLQKTTKSHQINSRQTILIIACCVGFVLMVLLFLAFLHLYFWDVWYIYHFCKAKIKGYQRLISPDCCYDAFIVYDTKDPAVTEWVLAELVAKLEDPREKHFNLCLEERDWLPGQPVLENLSQSIQLSKKTVFVMTDKYAKTENFKIAFYLSHQRLMDEKVDVIILIFLEKPFQKSKFLQLRKRLCGSSVLEWPTNPQAHPYFWQCLKNALATDNHVAYSQVFKETV

SEQ ID NO: 95 - skipped

SEQ ID NO: 96 - protein, 603 aa, Artificial Sequence
  CER30 chimeric engulfment receptor
  sig_peptide 1...22
MSKGLLLLWLVTELWWLYLTPAASEDTIIGFLGQPVTLPCHYLSWSQSRNSMCWGKGSCPNSKCNAELLRTDGTRIISRKSTKYTLLGKVQFGEVSLTISNTNRGDSGVYCCRIEVPGWFNDVKKNVRLELRRATTTKKPTTTTRPTTTPYVTTTTPELLPTTVMTTSVLPTTTPPQTLATTAFSTAVTTCPSTTPGSFSQETTKGSAFTTESETLPASNHSQRSMMTISTDIAVLRPTGSNPGILPSTSQLTTQKTTLTTSESLQKTTKSHQINSRQTILIIACCVGFVLMVLLFLAFLMAAASVTPPGSLELLQPGFSKTLLGTKLEAKYLCSACRNVLRRPFQAQCGHRYCSFCLASILSSGPQNCAACVHEGIYEEGISILESSSAFPDNAARREVESLPAVCPSDGCTWKGTLKEYESCHEGRCPLMLTECPACKGLVRLGEKERHLEHECPERSLSCRHCRAPCCGADVKAHHEVCPKFPLTCDGCGKKKIPREKFQDHVKTCGKCRVPCRFHAIGCLETVEGEKQQEHEVQWLREHLAMLLSSVLEAKPLLGDQSHAGSELLQRCESLEKKTATFENIVCVLNREVERVAMTAEAC

SEQ ID NO: 97 - protein, 574 aa, Artificial Sequence
  CER31 chimeric engulfment receptor
  sig_peptide 1...22
MSKGLLLLWLVTELWWLYLTPAASEDTIIGFLGQPVTLPCHYLSWSQSRNSMCWGKGSCPNSKCNAELLRTDGTRIISRKSTKYTLLGKVQFGEVSLTISNTNRGDSGVYCCRIEVPGWFNDVKKNVRLELRRATTTKKPTTTTRPTTTPYVTTTTPELLPTTVMTTSVLPTTTPPQTLATTAFSTAVTTCPSTTPGSFSQETTKGSAFTTESETLPASNHSQRSMMTISTDIAVLRPTGSNPGILPSTSQLTTQKTTLTTSESLQKTTKSHQINSRQTILIIACCVGFVLMVLLFLAFLMESSKKMDSPGALQTNPPLKLHTDRSAGTPVFVPEQGGYKEKFVKTVEDKYKCEKCHLVLCSPKQTECGHRFCESCMAALLSSSSPKCTACQESIVKDKVFKDNCCKREILALQIYCRNESRGCAEQLMLGHLLVHLKNDCHFEELPCVRPDCKEKVLRKDLRDHVEKACKYREATCSHCKSQVPMIALQKHEDTDCPCVVVSCPHKCSVQTLLRSELSAHLSECVNAPSTCSFKRYGCVFQGTNQQIKAHEASSAVQHVNLLKEWSNSLEKKV

SEQ ID NO: 98 - protein, 478 aa, Artificial Sequence
  CER42 chimeric engulfment receptor
  sig_peptide 1...22
MLLLVTSLLLCELPHPAFLLIPQVQLQQSGPGLVKPSQTLSLTCAISGDSVSSNSAAWNWIRQSPSRGLEWLGRTYYRSKWYNDYAVSVKSRITINPDTSKNQFSLQLNSVTPEDTAVYYCAREVTGDLEDAFDIWGQGTMVTVSSGGGGSDIQMTQSPSSLSASVGDRVTITCRASQTIWSYLNWYQQRPGKAPNLLIYAASSLQSGVPSRFSGRGSGTDFTLTISSLQAEDFATYYCQQSYSIPQTFGQGTKLEIKESKYGPPCPPCPTIIGVSVLSVLVVSVVAVLVYKFYFHLMLLAGCIKYGRGENIYDAFVIYSSQDEDWVRNELVKNLEEGVPPFQLCLHYRDFIPGVAIAANIIHEGFHKSRKVIVVVSQHFIQSRWCIFEYEIAQTWQFLSSRAGIIFIVLQKVEKTLLRQQVELYRLLSRNTYLEWEDSVLGRHIFWRRLRKALLDGKSWNPEGTVGTGCNWQEATSI

SEQ ID NO: 99 - protein, 22 aa, Homo sapiens
  GM-CSF signal peptide sequence
MLLLVTSLLLCELPHPAFLLIP

SEQ ID NO: 100 - protein, 22 aa, Mus musculus
  Tim4 signal peptide sequence
MSKGLLLLWLVTELWWLYLTPA

SEQ ID NO: 101 - protein, 19 aa, Artificial Sequence
  P2A self-cleaving peptide
ATNFSLLKQAGDVEENPGP

SEQ ID NO: 102 - protein, 18 aa, Artificial Sequence
  T2A self-cleaving peptide
EGRGSLLTCGDVEENPGP

SEQ ID NO: 103 - protein, 20 aa, Artificial Sequence
  E2A self-cleaving peptide
QCTNYALLKLAGDVESNPGP

SEQ ID NO: 104 - protein, 22 aa, Artificial Sequence
  F2A self-cleaving peptide
VKQTLNFDLLKLAGDVESNPGP

SEQ ID NO: 105 - protein, 285 aa, Homo sapiens
  truncated EGFR
RKVCNGIGIGEFKDSLSINATNIKHFKNCTSISGDLHILPVAFRGDSFTHTPPLDPQELDILKTVKEITGFLLIQAWPENRTDLHAFENLEIIRGRTKQHGQFSLAVVSLNITSLGLRSLKEISDGDVIISGNKNLCYANTINWKKLFGTSGQKTKIISNRGENSCKATGQVCHALCSPEGCWGPEPRDCVSCRNVSRGRECVDKCNLLEGEPREFVENSECIQCHPECLPQAMNITCTGRGPDNCIQCAHYIDGPHCVKTCPAGVMGENNTLVWKYADAGHVCH

SEQ ID NO: 106 - protein, 279 aa, Mus musculus
  Tim4 binding domain
  sig_peptide 1...22
MSKGLLLLWLVTELWWLYLTPAASEDTIIGFLGQPVTLPCHYLSWSQSRNSMCWGKGSCPNSKCNAELLRTDGTRIISRKSTKYTLLGKVQFGEVSLTISNTNRGDSGVYCCRIEVPGWFNDVKKNVRLELRRATTTKKPTTTTRPTTTPYVTTTTPELLPTTVMTTSVLPTTTPPQTLATTAFSTAVTTCPSTTPGSFSQETTKGSAFTTESETLPASNHSQRSMMTISTDIAVLRPTGSNPGILPSTSQLTTQKTTLTTSESLQKTTKSHQINSRQT

SEQ ID NO: 107 - protein, 257 aa, Mus musculus
  Tim4 binding domain without signal peptide
ASEDTIIGFLGQPVTLPCHYLSWSQSRNSMCWGKGSCPNSKCNAELLRTDGTRIISRKSTKYTLLGKVQFGEVSLTISNTNRGDSGVYCCRIEVPGWFNDVKKNVRLELRRATTTKKPTTTTRPTTTPYVTTTTPELLPTTVMTTSVLPTTTPPQTLATTAFSTAVTTCPSTTPGSFSQETTKGSAFTTESETLPASNHSQRSMMTISTDIAVLRPTGSNPGILPSTSQLTTQKTTLTTSESLQKTTKSHQINSRQT

SEQ ID NO: 108 - protein, 21 aa, Mus musculus
  Tim4 transmembrane domain
ILIIACCVGFVLMVLLFLAFL

SEQ ID NO: 109 - protein, 267 aa, Artificial Sequence
  FMC63 scFv
  sig_peptide 1...22
MLLLVTSLLLCELPHPAFLLIPDIQMTQTTSSLSASLGDRVTISCRASQDISKYLNWYQQKPDGTVKLLIYHTSRLHSGVPSRFSGSGSGTDYSLTISNLEQEDIATYFCQQGNTLPYTFGGGTKLEITGSTSGSGKPGSGEGSTKGEVKLQESGPGLVAPSQSLSVTCTVSGVSLPDYGVSWIRQPPRKGLEWLGVIWGSETTYYNSALKSRLTIIKDNSKSQVFLKMNSLQTDDTAIYYCAKHYYYGGSYAMDYWGQGTSVTVSS

SEQ ID NO: 110 - DNA, 81 bp, Homo sapiens
  misc_feature: CD28 transmembrane domain
ttttgggtgctggtggtggttggtggagtcctggcttgctatagcttgctagtaacagtggcctttattattttctgggtg

SEQ ID NO: 111 - DNA, 63 bp, Homo sapiens
  misc_feature: DAP12 transmembrane domain
ggcgtgctggcagggatcgtgatgggagacctggtgctgacagtgctcattgccctggccgtg

SEQ ID NO: 112 - DNA, 63 bp, Homo sapiens
  misc_feature: TLR4 transmembrane domain
accatcattggtgtgtcggtcctcagtgtgcttgtagtatctgttgtagcagttctggtctat

SEQ ID NO: 113 - DNA, 63 bp, Homo sapiens
  misc_feature: BAI1 transmembrane domain
gtgacgctcatcgtgggctgtggcgtgtcctctctcaccctgctcatgctggtcatcatctac

SEQ ID NO: 114 - protein, 24 aa, Homo sapiens
  VARIANT: Tim4 signal peptide
MSKEPLILWLMIEFWWLYLTPVTS

SEQ ID NO: 115 - DNA, 126 bp, Homo sapiens
  misc_feature: FcepsilonRIgamma signaling domain
cgactgaagatccaagtgcgaaaggcagctataaccagctatgagaaatcagatggtgtttacacgggcctgagcaccaggaaccaggagacttacgagactctgaagcatgagaaaccaccacag

SEQ ID NO: 116 - DNA, 156 bp, Homo sapiens
  misc_feature: DAP12 signaling domain
tattttctgggaaggctcgttcctagaggtagaggtgctgccgaagcagcgacgcgcaaacagaggattactgaaacggagtctccctaccaagagctgcaaggccagaggtcagatgtctattcagacttgaacacacaaaggccatactacaaa

SEQ ID NO: 117 - DNA, 255 bp, Homo sapiens
  misc_feature: BAFFR signaling domain
tcctggagacggcgacaaaggcgcttgcgcggcgcatcatccgcagaggcgcccgacggcgataaggacgcgcccgaaccccttgataaagttattatcttgtcaccgggaatttctgacgctacggcacccgcgtggcctcctccgggcgaagatcctggtacgacaccccctggacacagtgttcccgtgcccgcgacagagctcggtagcacagaactggtgaccacaaagacggcgggaccggaacagcaa

SEQ ID NO: 118 - DNA, 135 bp, Homo sapiens
  misc_feature: CD79b signaling domain
gacagtaaagccgggatggaagaggaccacacatacgaggggcttgacatagatcaaacagcgacatacgaagacatcgtaaccttgcggactggagaggttaaatggtcagtcggagaacaccccggccaagaa

SEQ ID NO: 119 - DNA, 258 bp, Homo sapiens
  misc_feature: NFAM1 signaling domain
ctctggaataaaaagaggatgcgcggcccgggaaaagacccaacgagaaagtgtcccgatccccgcagtgcgtcaagccccaagcagcatccttccgaaagcgtatatacggcacttcaacgccgggaaacggaggtatatgcgtgtattgagaacgaggacgggtcatccccgaccgccaaacagtcccctctcagccaagagcgacctcacaggtttgaggacgatggtgaactcaatctggtctacgaaaacctg

SEQ ID NO: 120 - DNA, 2754 bp, Homo sapiens
  misc_feature: BAI1 binding domain
gccgccggagcagacgcggggcccgggcccgagccgtgcgccacgctggtgcagggaaagttcttcggctacttctccgcggccgccgtgttcccggccaacgcctcgcgctgctcctggacgctacgcaacccggacccgcggcgctacactctctacatgaaggtggccaaggcgcccgtgccctgcagcggccccggccgcgtgcgcacctaccagttcgactccttcctcgagtccacgcgcacctacctgggcgtggagagcttcgacgaggtgctgcggctctgcgacccctccgcacccctggccttcctgcaggccagcaagcagttcctgcagatgcggcgccagcagccgccccagcacgacgggctccggccccgggccgggccgccgggccccaccgacgacttctccgtggagtacctggtggtggggaaccgcaaccccagccgtgccgcctgccagatgctgtgccgctggctggacgcgtgtctggccggtagtcgcagctcgcacccctgcgggatcatgcagaccccctgcgcctgcctgggcggcgaggcgggcggccctgccgcgggacccctggccccccgcggggatgtctgcttgagagatgcggtggctggtggccctgaaaactgcctcaccagcctgacccaggaccggggcgggcacggcgccacaggcggctggaagctgtggtccctgtggggcgaatgcacgcgggactgcgggggaggcctccagacgcggacgcgcacctgcctgcccgcgccgggcgtggagggcggcggctgcgagggggtgctggaggagggtcgccagtgcaaccgcgaggcctgcggccccgctgggcgcaccagctcccggagccagtccctgcggtccacagatgcccggcggcgcgaggagctgggggacgagctgcagcagtttgggttcccagccccccagaccggtgacccagcagccgaggagtggtccccgtggagcgtgtgctccagcacctgcggcgagggctggcagacccgcacgcgcttctgcgtgtcctcctcctacagcacgcagtgcagcggacccctgcgcgagcagcggctgtgcaacaactctgccgtgtgcccagtgcatggtgcctgggatgagtggtcgccctggagcctctgctccagcacctgtggccgtggctttcgggatcgcacgcgcacctgcaggcccccccagtttgggggcaacccctgtgagggccctgagaagcaaaccaagttctgcaacattgccctgtgccctggccgggcagtggatggaaactggaatgagtggtcgagctggagcgcctgctccgccagctgctcccagggccgacagcagcgcacgcgtgaatgcaacgggccttcctacgggggtgcggagtgccagggccactgggtggagacccgagactgcttcctgcagcagtgcccagtggatggcaagtggcaggcctgggcgtcatggggcagttgcagcgtcacgtgtggggctggcagccagcgacgggagcgtgtctgctctgggcccttcttcgggggagcagcctgccagggcccccaggatgagtaccggcagtgcggcacccagcggtgtcccgagccccatgagatctgtgatgaggacaactttggtgctgtgatctggaaggagaccccagcgggagaggtggctgctgtccggtgtccccgcaacgccacaggactcatcctgcgacggtgtgagctggacgaggaaggcatcgcctactgggagccccccacctacatccgctgtgtttccattgactacagaaacatccagatgatgacccgggagcacctggccaaggctcagcgagggctgcctggggagggggtctcggaggtcatccagacactggtggagatctctcaggacgggaccagctacagtggggacctgctgtccaccatcgatgtcctgaggaacatgacagagattttccggagagcgtactacagccccacccctggggacgtacagaactttgtccagatccttagcaacctgttggcagaggagaatcgggacaagtgggaggaggcccagctggcgggccccaacgccaaggagctgttccggctggtggaggactttgtggacgtcatcggcttccgcatgaaggacctgagggatgcataccaggtgacagacaacctggttctcagcatccataagctcccagccagcggagccactgacatcagcttccccatgaagggctggcgggccacgggtgactgggccaaggtgccagaggacagggtcactgtgtccaagagtgtcttctccacggggctgacagaggccgatgaagcatccgtgtttgtggtgggcaccgtgctctacaggaacctgggcagcttcctggccctgcagaggaacacgaccgtcctgaattctaaggtgatctccgtgactgtgaaacccccgcctcgctccctgcgcacacccttggagatcgagtttgcccacatgtataatggcaccaccaaccagacctgtatcctgtgggatgagacggatgtaccctcctcctccgcccccccgcagctcgggccctggtcgtggcgcggctgccgcacggtgcccctcgacgccctccggacgcgctgcctctgtgaccggctctccaccttcgccatcttagcccagctcagcgccgacgcgaacatggagaaggcgactctgccgtcg

SEQ ID NO: 121 - DNA, 63 bp, Homo sapiens
  misc_feature: FcepsilonRIgamma transmembrane domain
ctttgttacattctcgacgcgatattgttcctttatggaatagttttgacgctcctttattgc

SEQ ID NO: 122 - protein, 488 aa, Artificial Sequence
  CER43 chimeric engulfment receptor
  sig_peptide 1...22
MLLLVTSLLLCELPHPAFLLIPDIQMTQTTSSLSASLGDRVTISCRASQDISKYLNWYQQKPDGTVKLLIYHTSRLHSGVPSRFSGSGSGTDYSLTISNLEQEDIATYFCQQGNTLPYTFGGGTKLEITGSTSGSGKPGSGEGSTKGEVKLQESGPGLVAPSQSLSVTCTVSGVSLPDYGVSWIRQPPRKGLEWLGVIWGSETTYYNSALKSRLTIIKDNSKSQVFLKMNSLQTDDTAIYYCAKHYYYGGSYAMDYWGQGTSVTVSSPVLSLNITCQMNKTIIGVSVLSVLVVSVVAVLVYKFYFHLMLLAGCIKYGRGENIYDAFVIYSSQDEDWVRNELVKNLEEGVPPFQLCLHYRDFIPGVAIAANIIHEGFHKSRKVIVVVSQHFIQSRWCIFEYEIAQTWQFLSSRAGIIFIVLQKVEKTLLRQQVELYRLLSRNTYLEWEDSVLGRHIFWRRLRKALLDGKSWNPEGTVGTGCNWQEATSI

SEQ ID NO: 123 - protein, 487 aa, Artificial Sequence
  CER44 chimeric engulfment receptor
  sig_peptide 1...22
MLLLVTSLLLCELPHPAFLLIPDIQMTQTTSSLSASLGDRVTISCRASQDISKYLNWYQQKPDGTVKLLIYHTSRLHSGVPSRFSGSGSGTDYSLTISNLEQEDIATYFCQQGNTLPYTFGGGTKLEITGSTSGSGKPGSGEGSTKGEVKLQESGPGLVAPSQSLSVTCTVSGVSLPDYGVSWIRQPPRKGLEWLGVIWGSETTYYNSALKSRLTIIKDNSKSQVFLKMNSLQTDDTAIYYCAKHYYYGGSYAMDYWGQGTSVTVSSESKYGPPCPPCPTIIGVSVLSVLVVSVVAVLVYKFYFHLMLLAGCIKYGRGENIYDAFVIYSSQDEDWVRNELVKNLEEGVPPFQLCLHYRDFIPGVAIAANIIHEGFHKSRKVIVVVSQHFIQSRWCIFEYEIAQTWQFLSSRAGIIFIVLQKVEKTLLRQQVELYRLLSRNTYLEWEDSVLGRHIFWRRLRKALLDGKSWNPEGTVGTGCNWQEATSI

SEQ ID NO: 124 - protein, 574 aa, Artificial Sequence
  CER29 chimeric engulfment receptor
  sig_peptide 1...22
MSKGLLLLWLVTELWWLYLTPAASEDTIIGFLGQPVTLPCHYLSWSQSRNSMCWGKGSCPNSKCNAELLRTDGTRIISRKSTKYTLLGKVQFGEVSLTISNTNRGDSGVYCCRIEVPGWFNDVKKNVRLELRRATTTKKPTTTTRPTTTPYVTTTTPELLPTTVMTTSVLPTTTPPQTLATTAFSTAVTTCPSTTPGSFSQETTKGSAFTTESETLPASNHSQRSMMTISTDIAVLRPTGSNPGILPSTSQLTTQKTTLTTSESLQKTTKSHQINSRQTILIIACCVGFVLMVLLFLAFLMSLLNCENSCGSSQSESDCCVAMASSCSAVTKDDSVGGTASTGNLSSSFMEEIQGYDVEFDPPLESKYECPICLMALREAVQTPCGHRFCKACIIKSIRDAGHKCPVDNEILLENQLFPDNFAKREILSLMVKCPNEGCLHKMELRHLEDHQAHCEFALMDCPQCQRPFQKFHINIHILKDCPRRQVSCDNCAASMAFEDKEIHDQNCPLANVICEYCNTILIREQMPNHYDLDCPTAPIPCTFSTFGCHEKMQRNHLARHLQENTQSHMRMLA

SEQ ID NO: 125 - protein, 626 aa, Artificial Sequence
  CER110 chimeric engulfment receptor
  sig_peptide 1...22
MSKGLLLLWLVTELWWLYLTPAASEDTIIGFLGQPVTLPCHYLSWSQSRNSMCWGKGSCPNSKCNAELLRTDGTRIISRKSTKYTLLGKVQFGEVSLTISNTNRGDSGVYCCRIEVPGWFNDVKKNVRLELRRATTTKKPTTTTRPTTTPYVTTTTPELLPTTVMTTSVLPTTTPPQTLATTAFSTAVTTCPSTTPGSFSQETTKGSAFTTESETLPASNHSQRSMMTISTDIAVLRPTGSNPGILPSTSQLTTQKTTLTTSESLQKTTKSHQINSRQTILIIACCVGFVLMVLLFLAFLMSLLNCENSCGSSQSESDCCVAMASSCSAVTKDDSVGGTASTGNLSSSFMEEIQGYDVEFDPPLESKYECPICLMALREAVQTPCGHRFCKACIIKSIRDAGHKCPVDNEILLENQLFPDNFAKREILSLMVKCPNEGCLHKMELRHLEDHQAHCEFALMDCPQCQRPFQKFHINIHILKDCPRRQVSCDNCAASMAFEDKEIHDQNCPLANVICEYCNTILIREQMPNHYDLDCPTAPIPCTFSTFGCHEKMQRNHLARHLQENTQSHMRMLAYFLGRLVPRGRGAAEAATRKQRITETESPYQELQGQRSDVYSDLNTQRPYYK

SEQ ID NO: 126 - protein, 574 aa, Artificial Sequence; identical to SEQ ID NO: 124
  CER111B chimeric engulfment receptor
  sig_peptide 1...22

SEQ ID NO: 127 - protein, 638 aa, Artificial Sequence
  CER113 chimeric engulfment receptor
  sig_peptide 1...22
MSKGLLLLWLVTELWWLYLTPAASEDTIIGFLGQPVTLPCHYLSWSQSRNSMCWGKGSCPNSKCNAELLRTDGTRIISRKSTKYTLLGKVQFGEVSLTISNTNRGDSGVYCCRIEVPGWFNDVKKNVRLELRRATTTKKPTTTTRPTTTPYVTTTTPELLPTTVMTTSVLPTTTPPQTLATTAFSTAVTTCPSTTPGSFSQETTKGSAFTTESETLPASNHSQRSMMTISTDIAVLRPTGSNPGILPSTSQLTTQKTTLTTSESLQKTTKSHQINSRQTMSLLNCENSCGSSQSESDCCVAMASSCSAVTKDDSVGGTASTGNLSSSFMEEIQGYDVEFDPPLESKYECPICLMALREAVQTPCGHRFCKACIIKSIRDAGHKCPVDNEILLENQLFPDNFAKREILSLMVKCPNEGCLHKMELRHLEDHQAHCEFALMDCPQCQRPFQKFHINIHILKDCPRRQVSCDNCAASMAFEDKEIHDQNCPLANVICEYCNTILIREQMPNHYDLDCPTAPIPCTFSTFGCHEKMQRNHLARHLQENTQSHMRMLASWRRRQRRLRGASSAEAPDGDKDAPEPLDKVIILSPGISDATAPAWPPPGEDPGTTPPGHSVPVPATELGSTELVTTKTAGPEQQ

SEQ ID NO: 128 - protein, 660 aa, Artificial Sequence
  CER112 chimeric engulfment receptor
  sig_peptide 1...22
MSKGLLLLWLVTELWWLYLTPAASEDTIIGFLGQPVTLPCHYLSWSQSRNSMCWGKGSCPNSKCNAELLRTDGTRIISRKSTKYTLLGKVQFGEVSLTISNTNRGDSGVYCCRIEVPGWFNDVKKNVRLELRRATTTKKPTTTTRPTTTPYVTTTTPELLPTTVMTTSVLPTTTPPQTLATTAFSTAVTTCPSTTPGSFSQETTKGSAFTTESETLPASNHSQRSMMTISTDIAVLRPTGSNPGILPSTSQLTTQKTTLTTSESLQKTTKSHQINSRQTILIIACCVGFVLMVLLFLAFLMSLLNCENSCGSSQSESDCCVAMASSCSAVTKDDSVGGTASTGNLSSSFMEEIQGYDVEFDPPLESKYECPICLMALREAVQTPCGHRFCKACIIKSIRDAGHKCPVDNEILLENQLFPDNFAKREILSLMVKCPNEGCLHKMELRHLEDHQAHCEFALMDCPQCQRPFQKFHINIHILKDCPRRQVSCDNCAASMAFEDKEIHDQNCPLANVICEYCNTILIREQMPNHYDLDCPTAPIPCTFSTFGCHEKMQRNHLARHLQENTQSHMRMLALWNKKRMRGPGKDPTRKCPDPRSASSPKQHPSESVYTALQRRETEVYACIENEDGSSPTAKQSPLSQERPHRFEDDGELNLVYENL

SEQ ID NO: 129 - skipped

SEQ ID NO: 130 - protein, 579 aa, Artificial Sequence
  CER102 protein
  sig_peptide 1...22
MSKGLLLLWLVTELWWLYLTPAASEDTIIGFLGQPVTLPCHYLSWSQSRNSMCWGKGSCPNSKCNAELLRTDGTRIISRKSTKYTLLGKVQFGEVSLTISNTNRGDSGVYCCRIEVPGWFNDVKKNVRLELRRATTTKKPTTTTRPTTTPYVTTTTPELLPTTVMTTSVLPTTTPPQTLATTAFSTAVTTCPSTTPGSFSQETTKGSAFTTESETLPASNHSQRSMMTISTDIAVLRPTGSNPGILPSTSQLTTQKTTLTTSESLQKTTKSHQINSRQTILIIACCVGFVLMVLLFLAFLHHLFYWDVWFIYNVCLAKVKGYRSLSTSQTFYDAYISYDTKDASVTDWVINELRYHLEESRDKNVLLCLEERDWDPGLAIIDNLMQSINQSKKTVFVLTKKYAKSWNFKTAFYLALQRLMDENMDVIIFILLEPVLQHSQYLRLRQRICKSSILQWPDNPKAEGLFWQTLRNVVLTENDSRYNNMYVDSIKQYLWNKKRMRGPGKDPTRKCPDPRSASSPKQHPSESVYTALQRRETEVYACIENEDGSSPTAKQSPLSQERPHRFEDDGELNLVYENL

SEQ ID NO: 131 - protein, 538 aa, Artificial Sequence
  CER103A protein
  sig_peptide 1...22
MSKGLLLLWLVTELWWLYLTPAASEDTIIGFLGQPVTLPCHYLSWSQSRNSMCWGKGSCPNSKCNAELLRTDGTRIISRKSTKYTLLGKVQFGEVSLTISNTNRGDSGVYCCRIEVPGWFNDVKKNVRLELRRATTTKKPTTTTRPTTTPYVTTTTPELLPTTVMTTSVLPTTTPPQTLATTAFSTAVTTCPSTTPGSFSQETTKGSAFTTESETLPASNHSQRSMMTISTDIAVLRPTGSNPGILPSTSQLTTQKTTLTTSESLQKTTKSHQINSRQTILIIACCVGFVLMVLLFLAFLHHLFYWDVWFIYNVCLAKVKGYRSLSTSQTFYDAYISYDTKDASVTDWVINELRYHLEESRDKNVLLCLEERDWDPGLAIIDNLMQSINQSKKTVFVLTKKYAKSWNFKTAFYLALQRLMDENMDVIIFILLEPVLQHSQYLRLRQRICKSSILQWPDNPKAEGLFWQTLRNVVLTENDSRYNNMYVDSIKQYDSKAGMEEDHTYEGLDIDQTATYEDIVTLRTGEVKWSVGEHPGQE

SEQ ID NO: 132 - protein, 522 aa, Artificial Sequence
  CER103B protein
  sig_peptide 1...22
MSKGLLLLWLVTELWWLYLTPAASEDTIIGFLGQPVTLPCHYLSWSQSRNSMCWGKGSCPNSKCNAELLRTDGTRIISRKSTKYTLLGKVQFGEVSLTISNTNRGDSGVYCCRIEVPGWFNDVKKNVRLELRRATTTKKPTTTTRPTTTPYVTTTTPELLPTTVMTTSVLPTTTPPQTLATTAFSTAVTTCPSTTPGSFSQETTKGSAFTTESETLPASNHSQRSMMTISTDIAVLRPTGSNPGILPSTSQLTTQKTTLTTSESLQKTTKSHQINSRQTILIIACCVGFVLMVLLFLAFLHHLFYWDVWFIYNVCLAKVKGYRSLSTSQTFYDAYISYDTKDASVTDWVINELRYHLEESRDKNVLLCLEERDWDPGLAIIDNLMQSINQSKKTVFVLTKKYAKSWNFKTAFYLALQRLMDENMDVIIFILLEPVLQHSQYLRLRQRICKSSILQWPDNPKAEGLFWQTLRNVVLTENDSRYNNMYVDSIKQYDSKAGMEEDHTYEGLDIDQTATYEDIVTL

SEQ ID NO: 133 - protein, 545 aa, Artificial Sequence
  CER104 protein
  sig_peptide 1...22
MSKGLLLLWLVTELWWLYLTPAASEDTIIGFLGQPVTLPCHYLSWSQSRNSMCWGKGSCPNSKCNAELLRTDGTRIISRKSTKYTLLGKVQFGEVSLTISNTNRGDSGVYCCRIEVPGWFNDVKKNVRLELRRATTTKKPTTTTRPTTTPYVTTTTPELLPTTVMTTSVLPTTTPPQTLATTAFSTAVTTCPSTTPGSFSQETTKGSAFTTESETLPASNHSQRSMMTISTDIAVLRPTGSNPGILPSTSQLTTQKTTLTTSESLQKTTKSHQINSRQTILIIACCVGFVLMVLLFLAFLHHLFYWDVWFIYNVCLAKVKGYRSLSTSQTFYDAYISYDTKDASVTDWVINELRYHLEESRDKNVLLCLEERDWDPGLAIIDNLMQSINQSKKTVFVLTKKYAKSWNFKTAFYLALQRLMDENMDVIIFILLEPVLQHSQYLRLRQRICKSSILQWPDNPKAEGLFWQTLRNVVLTENDSRYNNMYVDSIKQYYFLGRLVPRGRGAAEAATRKQRITETESPYQELQGQRSDVYSDLNTQRPYYK

SEQ ID NO: 134 - protein, 578 aa, Artificial Sequence
  CER105 protein
  sig_peptide 1...22
MSKGLLLLWLVTELWWLYLTPAASEDTIIGFLGQPVTLPCHYLSWSQSRNSMCWGKGSCPNSKCNAELLRTDGTRIISRKSTKYTLLGKVQFGEVSLTISNTNRGDSGVYCCRIEVPGWFNDVKKNVRLELRRATTTKKPTTTTRPTTTPYVTTTTPELLPTTVMTTSVLPTTTPPQTLATTAFSTAVTTCPSTTPGSFSQETTKGSAFTTESETLPASNHSQRSMMTISTDIAVLRPTGSNPGILPSTSQLTTQKTTLTTSESLQKTTKSHQINSRQTILIIACCVGFVLMVLLFLAFLHHLFYWDVWFIYNVCLAKVKGYRSLSTSQTFYDAYISYDTKDASVTDWVINELRYHLEESRDKNVLLCLEERDWDPGLAIIDNLMQSINQSKKTVFVLTKKYAKSWNFKTAFYLALQRLMDENMDVIIFILLEPVLQHSQYLRLRQRICKSSILQWPDNPKAEGLFWQTLRNVVLTENDSRYNNMYVDSIKQYSWRRRQRRLRGASSAEAPDGDKDAPEPLDKVIILSPGISDATAPAWPPPGEDPGTTPPGHSVPVPATELGSTELVTTKTAGPEQQ

SEQ ID NO: 135 - protein, 579 aa, Artificial Sequence
  CER106 protein
  sig_peptide 1...22
MSKGLLLLWLVTELWWLYLTPAASEDTIIGFLGQPVTLPCHYLSWSQSRNSMCWGKGSCPNSKCNAELLRTDGTRIISRKSTKYTLLGKVQFGEVSLTISNTNRGDSGVYCCRIEVPGWFNDVKKNVRLELRRATTTKKPTTTTRPTTTPYVTTTTPELLPTTVMTTSVLPTTTPPQTLATTAFSTAVTTCPSTTPGSFSQETTKGSAFTTESETLPASNHSQRSMMTISTDIAVLRPTGSNPGILPSTSQLTTQKTTLTTSESLQKTTKSHQINSRQTILIIACCVGFVLMVLLFLAFLLWNKKRMRGPGKDPTRKCPDPRSASSPKQHPSESVYTALQRRETEVYACIENEDGSSPTAKQSPLSQERPHRFEDDGELNLVYENLHHLFYWDVWFIYNVCLAKVKGYRSLSTSQTFYDAYISYDTKDASVTDWVINELRYHLEESRDKNVLLCLEERDWDPGLAIIDNLMQSINQSKKTVFVLTKKYAKSWNFKTAFYLALQRLMDENMDVIIFILLEPVLQHSQYLRLRQRICKSSILQWPDNPKAEGLFWQTLRNVVLTENDSRYNNMYVDSIKQY

SEQ ID NO: 136 - protein, 522 aa, Artificial Sequence
  CER107 protein
  sig_peptide 1...22
MSKGLLLLWLVTELWWLYLTPAASEDTIIGFLGQPVTLPCHYLSWSQSRNSMCWGKGSCPNSKCNAELLRTDGTRIISRKSTKYTLLGKVQFGEVSLTISNTNRGDSGVYCCRIEVPGWFNDVKKNVRLELRRATTTKKPTTTTRPTTTPYVTTTTPELLPTTVMTTSVLPTTTPPQTLATTAFSTAVTTCPSTTPGSFSQETTKGSAFTTESETLPASNHSQRSMMTISTDIAVLRPTGSNPGILPSTSQLTTQKTTLTTSESLQKTTKSHQINSRQTILIIACCVGFVLMVLLFLAFLDSKAGMEEDHTYEGLDIDQTATYEDIVTLHHLFYWDVWFIYNVCLAKVKGYRSLSTSQTFYDAYISYDTKDASVTDWVINELRYHLEESRDKNVLLCLEERDWDPGLAIIDNLMQSINQSKKTVFVLTKKYAKSWNFKTAFYLALQRLMDENMDVIIFILLEPVLQHSQYLRLRQRICKSSILQWPDNPKAEGLFWQTLRNVVLTENDSRYNNMYVDSIKQY

SEQ ID NO: 137 - protein, 545 aa, Artificial Sequence
  CER108 protein
  sig_peptide 1...22
MSKGLLLLWLVTELWWLYLTPAASEDTIIGFLGQPVTLPCHYLSWSQSRNSMCWGKGSCPNSKCNAELLRTDGTRIISRKSTKYTLLGKVQFGEVSLTISNTNRGDSGVYCCRIEVPGWFNDVKKNVRLELRRATTTKKPTTTTRPTTTPYVTTTTPELLPTTVMTTSVLPTTTPPQTLATTAFSTAVTTCPSTTPGSFSQETTKGSAFTTESETLPASNHSQRSMMTISTDIAVLRPTGSNPGILPSTSQLTTQKTTLTTSESLQKTTKSHQINSRQTILIIACCVGFVLMVLLFLAFLYFLGRLVPRGRGAAEAATRKQRITETESPYQELQGQRSDVYSDLNTQRPYYKHHLFYWDVWFIYNVCLAKVKGYRSLSTSQTFYDAYISYDTKDASVTDWVINELRYHLEESRDKNVLLCLEERDWDPGLAIIDNLMQSINQSKKTVFVLTKKYAKSWNFKTAFYLALQRLMDENMDVIIFILLEPVLQHSQYLRLRQRICKSSILQWPDNPKAEGLFWQTLRNVVLTENDSRYNNMYVDSIKQY

SEQ ID NO: 138 - protein, 578 aa, Artificial Sequence
  CER109 protein
  sig_peptide 1...22
MSKGLLLLWLVTELWWLYLTPAASEDTIIGFLGQPVTLPCHYLSWSQSRNSMCWGKGSCPNSKCNAELLRTDGTRIISRKSTKYTLLGKVQFGEVSLTISNTNRGDSGVYCCRIEVPGWFNDVKKNVRLELRRATTTKKPTTTTRPTTTPYVTTTTPELLPTTVMTTSVLPTTTPPQTLATTAFSTAVTTCPSTTPGSFSQETTKGSAFTTESETLPASNHSQRSMMTISTDIAVLRPTGSNPGILPSTSQLTTQKTTLTTSESLQKTTKSHQINSRQTILIIACCVGFVLMVLLFLAFLSWRRRQRRLRGASSAEAPDGDKDAPEPLDKVIILSPGISDATAPAWPPPGEDPGTTPPGHSVPVPATELGSTELVTTKTAGPEQQHHLFYWDVWFIYNVCLAKVKGYRSLSTSQTFYDAYISYDTKDASVTDWVINELRYHLEESRDKNVLLCLEERDWDPGLAIIDNLMQSINQSKKTVFVLTKKYAKSWNFKTAFYLALQRLMDENMDVIIFILLEPVLQHSQYLRLRQRICKSSILQWPDNPKAEGLFWQTLRNVVLTENDSRYNNMYVDSIKQY

SEQ ID NO: 139 - protein, 619 aa, Artificial Sequence
  CER111A protein
  sig_peptide 1...22
MSKGLLLLWLVTELWWLYLTPAASEDTIIGFLGQPVTLPCHYLSWSQSRNSMCWGKGSCPNSKCNAELLRTDGTRIISRKSTKYTLLGKVQFGEVSLTISNTNRGDSGVYCCRIEVPGWFNDVKKNVRLELRRATTTKKPTTTTRPTTTPYVTTTTPELLPTTVMTTSVLPTTTPPQTLATTAFSTAVTTCPSTTPGSFSQETTKGSAFTTESETLPASNHSQRSMMTISTDIAVLRPTGSNPGILPSTSQLTTQKTTLTTSESLQKTTKSHQINSRQTILIIACCVGFVLMVLLFLAFLMSLLNCENSCGSSQSESDCCVAMASSCSAVTKDDSVGGTASTGNLSSSFMEEIQGYDVEFDPPLESKYECPICLMALREAVQTPCGHRFCKACIIKSIRDAGHKCPVDNEILLENQLFPDNFAKREILSLMVKCPNEGCLHKMELRHLEDHQAHCEFALMDCPQCQRPFQKFHINIHILKDCPRRQVSCDNCAASMAFEDKEIHDQNCPLANVICEYCNTILIREQMPNHYDLDCPTAPIPCTFSTFGCHEKMQRNHLARHLQENTQSHMRMLADSKAGMEEDHTYEGLDIDQTATYEDIVTLRTGEVKWSVGEHPGQE

SEQ ID NO: 140 - protein, 659 aa, Artificial Sequence
  CER113 protein
  sig_peptide 1...22
MSKGLLLLWLVTELWWLYLTPAASEDTIIGFLGQPVTLPCHYLSWSQSRNSMCWGKGSCPNSKCNAELLRTDGTRIISRKSTKYTLLGKVQFGEVSLTISNTNRGDSGVYCCRIEVPGWFNDVKKNVRLELRRATTTKKPTTTTRPTTTPYVTTTTPELLPTTVMTTSVLPTTTPPQTLATTAFSTAVTTCPSTTPGSFSQETTKGSAFTTESETLPASNHSQRSMMTISTDIAVLRPTGSNPGILPSTSQLTTQKTTLTTSESLQKTTKSHQINSRQTILIIACCVGFVLMVLLFLAFLMSLLNCENSCGSSQSESDCCVAMASSCSAVTKDDSVGGTASTGNLSSSFMEEIQGYDVEFDPPLESKYECPICLMALREAVQTPCGHRFCKACIIKSIRDAGHKCPVDNEILLENQLFPDNFAKREILSLMVKCPNEGCLHKMELRHLEDHQAHCEFALMDCPQCQRPFQKFHINIHILKDCPRRQVSCDNCAASMAFEDKEIHDQNCPLANVICEYCNTILIREQMPNHYDLDCPTAPIPCTFSTFGCHEKMQRNHLARHLQENTQSHMRMLASWRRRQRRLRGASSAEAPDGDKDAPEPLDKVIILSPGISDATAPAWPPPGEDPGTTPPGHSVPVPATELGSTELVTTKTAGPEQQ

SEQ ID NO: 141 - protein, 1050 aa, Artificial Sequence
  CER114 protein
  sig_peptide 1...22
MSKGLLLLWLVTELWWLYLTPAASEDTIIGFLGQPVTLPCHYLSWSQSRNSMCWGKGSCPNSKCNAELLRTDGTRIISRKSTKYTLLGKVQFGEVSLTISNTNRGDSGVYCCRIEVPGWFNDVKKNVRLELRRATTTKKPTTTTRPTTTPYVTTTTPELLPTTVMTTSVLPTTTPPQTLATTAFSTAVTTCPSTTPGSFSQETTKGSAFTTESETLPASNHSQRSMMTISTDIAVLRPTGSNPGILPSTSQLTTQKTTLTTSESLQKTTKSHQINSRQTILIIACCVGFVLMVLLFLAFLMSLLNCENSCGSSQSESDCCVAMASSCSAVTKDDSVGGTASTGNLSSSFMEEIQGYDVEFDPPLESKYECPICLMALREAVQTPCGHRFCKACIIKSIRDAGHKCPVDNEILLENQLFPDNFAKREILSLMVKCPNEGCLHKMELRHLEDHQAHCEFALMDCPQCQRPFQKFHINIHILKDCPRRQVSCDNCAASMAFEDKEIHDQNCPLANVICEYCNTILIREQMPNHYDLDCPTAPIPCTFSTFGCHEKMQRNHLARHLQENTQSHMRMLAALRRRVQETKFGGAFSEEDSQLVVNYRAKKSFCRRAIELTLQSLGVSEELQNKLEDVVIDRNLLVLGKVLGEGEFGSVMEGNLKQEDGTSQKVAVKTMKLDNFSQREIEEFLSEAACMKDFNHPNVIRLLGVCIELSSQGIPKPMVILPFMKYGDLHTFLLYSRLNTGPKYIHLQTLLKFMMDIAQGMEYLSNRNFLHRDLAARNCMLRDDMTVCVADFGLSKKIYSGDYYRQGRIAKMPVKWIAIESLADRVYTSKSDVWAFGVTMWEITTRGMTPYPGVQNHEMYDYLLHGHRLKQPEDCLDELYDIMYSCWSADPLDRPTFSVLRLQLEKLSESLPDAQDKESIIYINTQLLESCEGIANGPSLTGLDMNIDPDSIIASCTPGAAVSVVTAEVHENNLREERYILNGGNEEWEDVSSTPFAAVTPEKDGVLPEDRLTKNGVSWSHHSTLPLGSPSPDELLFVDDSLEDSEVLM

SEQ ID NO: 142 - protein, 1050 aa, Artificial Sequence
  CER115 protein
  sig_peptide 1...22
MSKGLLLLWLVTELWWLYLTPAASEDTIIGFLGQPVTLPCHYLSWSQSRNSMCWGKGSCPNSKCNAELLRTDGTRIISRKSTKYTLLGKVQFGEVSLTISNTNRGDSGVYCCRIEVPGWFNDVKKNVRLELRRATTTKKPTTTTRPTTTPYVTTTTPELLPTTVMTTSVLPTTTPPQTLATTAFSTAVTTCPSTTPGSFSQETTKGSAFTTESETLPASNHSQRSMMTISTDIAVLRPTGSNPGILPSTSQLTTQKTTLTTSESLQKTTKSHQINSRQTILIIACCVGFVLMVLLFLAFLALRRRVQETKFGGAFSEEDSQLVVNYRAKKSFCRRAIELTLQSLGVSEELQNKLEDVVIDRNLLVLGKVLGEGEFGSVMEGNLKQEDGTSQKVAVKTMKLDNFSQREIEEFLSEAACMKDFNHPNVIRLLGVCIELSSQGIPKPMVILPFMKYGDLHTFLLYSRLNTGPKYIHLQTLLKFMMDIAQGMEYLSNRNFLHRDLAARNCMLRDDMTVCVADFGLSKKIYSGDYYRQGRIAKMPVKWIAIESLADRVYTSKSDVWAFGVTMWEITTRGMTPYPGVQNHEMYDYLLHGHRLKQPEDCLDELYDIMYSCWSADPLDRPTFSVLRLQLEKLSESLPDAQDKESIIYINTQLLESCEGIANGPSLTGLDMNIDPDSIIASCTPGAAVSVVTAEVHENNLREERYILNGGNEEWEDVSSTPFAAVTPEKDGVLPEDRLTKNGVSWSHHSTLPLGSPSPDELLFVDDSLEDSEVLMMSLLNCENSCGSSQSESDCCVAMASSCSAVTKDDSVGGTASTGNLSSSFMEEIQGYDVEFDPPLESKYECPICLMALREAVQTPCGHRFCKACIIKSIRDAGHKCPVDNEILLENQLFPDNFAKREILSLMVKCPNEGCLHKMELRHLEDHQAHCEFALMDCPQCQRPFQKFHINIHILKDCPRRQVSCDNCAASMAFEDKEIHDQNCPLANVICEYCNTILIREQMPNHYDLDCPTAPIPCTFSTFGCHEKMQRNHLARHLQENTQSHMRMLA

SEQ ID NO: 143 - protein, 767 aa, Artificial Sequence
  CER116 protein
  sig_peptide 1...22
MSKGLLLLWLVTELWWLYLTPAASEDTIIGFLGQPVTLPCHYLSWSQSRNSMCWGKGSCPNSKCNAELLRTDGTRIISRKSTKYTLLGKVQFGEVSLTISNTNRGDSGVYCCRIEVPGWFNDVKKNVRLELRRATTTKKPTTTTRPTTTPYVTTTTPELLPTTVMTTSVLPTTTPPQTLATTAFSTAVTTCPSTTPGSFSQETTKGSAFTTESETLPASNHSQRSMMTISTDIAVLRPTGSNPGILPSTSQLTTQKTTLTTSESLQKTTKSHQINSRQTILIIACCVGFVLMVLLFLAFLMSLLNCENSCGSSQSESDCCVAMASSCSAVTKDDSVGGTASTGNLSSSFMEEIQGYDVEFDPPLESKYECPICLMALREAVQTPCGHRFCKACIIKSIRDAGHKCPVDNEILLENQLFPDNFAKREILSLMVKCPNEGCLHKMELRHLEDHQAHCEFALMDCPQCQRPFQKFHINIHILKDCPRRQVSCDNCAASMAFEDKEIHDQNCPLANVICEYCNTILIREQMPNHYDLDCPTAPIPCTFSTFGCHEKMQRNHLARHLQENTQSHMRMLAHHLFYWDVWFIYNVCLAKVKGYRSLSTSQTFYDAYISYDTKDASVTDWVINELRYHLEESRDKNVLLCLEERDWDPGLAIIDNLMQSINQSKKTVFVLTKKYAKSWNFKTAFYLALQRLMDENMDVIIFILLEPVLQHSQYLRLRQRICKSSILQWPDNPKAEGLFWQTLRNVVLTENDSRYNNMYVDSIKQY

SEQ ID NO: 144 - protein, 767 aa, Artificial Sequence
  CER117 protein
  sig_peptide 1...22
MSKGLLLLWLVTELWWLYLTPAASEDTIIGFLGQPVTLPCHYLSWSQSRNSMCWGKGSCPNSKCNAELLRTDGTRIISRKSTKYTLLGKVQFGEVSLTISNTNRGDSGVYCCRIEVPGWFNDVKKNVRLELRRATTTKKPTTTTRPTTTPYVTTTTPELLPTTVMTTSVLPTTTPPQTLATTAFSTAVTTCPSTTPGSFSQETTKGSAFTTESETLPASNHSQRSMMTISTDIAVLRPTGSNPGILPSTSQLTTQKTTLTTSESLQKTTKSHQINSRQTILIIACCVGFVLMVLLFLAFLHHLFYWDVWFIYNVCLAKVKGYRSLSTSQTFYDAYISYDTKDASVTDWVINELRYHLEESRDKNVLLCLEERDWDPGLAIIDNLMQSINQSKKTVFVLTKKYAKSWNFKTAFYLALQRLMDENMDVIIFILLEPVLQHSQYLRLRQRICKSSILQWPDNPKAEGLFWQTLRNVVLTENDSRYNNMYVDSIKQYMSLLNCENSCGSSQSESDCCVAMASSCSAVTKDDSVGGTASTGNLSSSFMEEIQGYDVEFDPPLESKYECPICLMALREAVQTPCGHRFCKACIIKSIRDAGHKCPVDNEILLENQLFPDNFAKREILSLMVKCPNEGCLHKMELRHLEDHQAHCEFALMDCPQCQRPFQKFHINIHILKDCPRRQVSCDNCAASMAFEDKEIHDQNCPLANVICEYCNTILIREQMPNHYDLDCPTAPIPCTFSTFGCHEKMQRNHLARHLQENTQSHMRMLA

SEQ ID NO: 145 - protein, 571 aa, Artificial Sequence
  CER118 protein
  sig_peptide 1...22
MSKGLLLLWLVTELWWLYLTPAASEDTIIGFLGQPVTLPCHYLSWSQSRNSMCWGKGSCPNSKCNAELLRTDGTRIISRKSTKYTLLGKVQFGEVSLTISNTNRGDSGVYCCRIEVPGWFNDVKKNVRLELRRATTTKKPTTTTRPTTTPYVTTTTPELLPTTVMTTSVLPTTTPPQTLATTAFSTAVTTCPSTTPGSFSQETTKGSAFTTESETLPASNHSQRSMMTISTDIAVLRPTGSNPGILPSTSQLTTQKTTLTTSESLQKTTKSHQINSRQTILIIACCVGFVLMVLLFLAFLSYLDLPWYLRMVCQWTQTRRRARNIPLEELQRNLQFHAFISYSGHDSFWVKNELLPNLEKEGMQICLHERNFVPGKSIVENIITCIEKSYKSIFVLSPNFVQSEWCHYELYFAHHNLFHEGSNSLILILLEPIPQYSIPSSYHKLKSLMARRTYLEWPKEKSKRGLFWANLRAAINIKLTEQAKKLWNKKRMRGPGKDPTRKCPDPRSASSPKQHPSESVYTALQRRETEVYACIENEDGSSPTAKQSPLSQERPHRFEDDGELNLVYENL

SEQ ID NO: 146 - protein, 514 aa, Artificial Sequence
  CER119B protein
  sig_peptide 1...22
MSKGLLLLWLVTELWWLYLTPAASEDTIIGFLGQPVTLPCHYLSWSQSRNSMCWGKGSCPNSKCNAELLRTDGTRIISRKSTKYTLLGKVQFGEVSLTISNTNRGDSGVYCCRIEVPGWFNDVKKNVRLELRRATTTKKPTTTTRPTTTPYVTTTTPELLPTTVMTTSVLPTTTPPQTLATTAFSTAVTTCPSTTPGSFSQETTKGSAFTTESETLPASNHSQRSMMTISTDIAVLRPTGSNPGILPSTSQLTTQKTTLTTSESLQKTTKSHQINSRQTILIIACCVGFVLMVLLFLAFLSYLDLPWYLRMVCQWTQTRRRARNIPLEELQRNLQFHAFISYSGHDSFWVKNELLPNLEKEGMQICLHERNFVPGKSIVENIITCIEKSYKSIFVLSPNFVQSEWCHYELYFAHHNLFHEGSNSLILILLEPIPQYSIPSSYHKLKSLMARRTYLEWPKEKSKRGLFWANLRAAINIKLTEQAKKDSKAGMEEDHTYEGLDIDQTATYEDIVTL

SEQ ID NO: 147 - protein, 537 aa, Artificial Sequence
  CER120 protein
  sig_peptide 1...22
MSKGLLLLWLVTELWWLYLTPAASEDTIIGFLGQPVTLPCHYLSWSQSRNSMCWGKGSCPNSKCNAELLRTDGTRIISRKSTKYTLLGKVQFGEVSLTISNTNRGDSGVYCCRIEVPGWFNDVKKNVRLELRRATTTKKPTTTTRPTTTPYVTTTTPELLPTTVMTTSVLPTTTPPQTLATTAFSTAVTTCPSTTPGSFSQETTKGSAFTTESETLPASNHSQRSMMTISTDIAVLRPTGSNPGILPSTSQLTTQKTTLTTSESLQKTTKSHQINSRQTILIIACCVGFVLMVLLFLAFLSYLDLPWYLRMVCQWTQTRRRARNIPLEELQRNLQFHAFISYSGHDSFWVKNELLPNLEKEGMQICLHERNFVPGKSIVENIITCIEKSYKSIFVLSPNFVQSEWCHYELYFAHHNLFHEGSNSLILILLEPIPQYSIPSSYHKLKSLMARRTYLEWPKEKSKRGLFWANLRAAINIKLTEQAKKYFLGRLVPRGRGAAEAATRKQRITETESPYQELQGQRSDVYSDLNTQRPYYK

SEQ ID NO: 148 - protein, 759 aa, Artificial Sequence
  CER121 protein
  sig_peptide 1...22
MSKGLLLLWLVTELWWLYLTPAASEDTIIGFLGQPVTLPCHYLSWSQSRNSMCWGKGSCPNSKCNAELLRTDGTRIISRKSTKYTLLGKVQFGEVSLTISNTNRGDSGVYCCRIEVPGWFNDVKKNVRLELRRATTTKKPTTTTRPTTTPYVTTTTPELLPTTVMTTSVLPTTTPPQTLATTAFSTAVTTCPSTTPGSFSQETTKGSAFTTESETLPASNHSQRSMMTISTDIAVLRPTGSNPGILPSTSQLTTQKTTLTTSESLQKTTKSHQINSRQTILIIACCVGFVLMVLLFLAFLSYLDLPWYLRMVCQWTQTRRRARNIPLEELQRNLQFHAFISYSGHDSFWVKNELLPNLEKEGMQICLHERNFVPGKSIVENIITCIEKSYKSIFVLSPNFVQSEWCHYELYFAHHNLFHEGSNSLILILLEPIPQYSIPSSYHKLKSLMARRTYLEWPKEKSKRGLFWANLRAAINIKLTEQAKKMSLLNCENSCGSSQSESDCCVAMASSCSAVTKDDSVGGTASTGNLSSSFMEEIQGYDVEFDPPLESKYECPICLMALREAVQTPCGHRFCKACIIKSIRDAGHKCPVDNEILLENQLFPDNFAKREILSLMVKCPNEGCLHKMELRHLEDHQAHCEFALMDCPQCQRPFQKFHINIHILKDCPRRQVSCDNCAASMAFEDKEIHDQNCPLANVICEYCNTILIREQMPNHYDLDCPTAPIPCTFSTFGCHEKMQRNHLARHLQENTQSHMRMLA

SEQ ID NO: 149 - protein, 527 aa, Artificial Sequence
  CER122 protein
  sig_peptide 1...22
MSKGLLLLWLVTELWWLYLTPAASEDTIIGFLGQPVTLPCHYLSWSQSRNSMCWGKGSCPNSKCNAELLRTDGTRIISRKSTKYTLLGKVQFGEVSLTISNTNRGDSGVYCCRIEVPGWFNDVKKNVRLELRRATTTKKPTTTTRPTTTPYVTTTTPELLPTTVMTTSVLPTTTPPQTLATTAFSTAVTTCPSTTPGSFSQETTKGSAFTTESETLPASNHSQRSMMTISTDIAVLRPTGSNPGILPSTSQLTTQKTTLTTSESLQKTTKSHQINSRQTILIIACCVGFVLMVLLFLAFLHRFHGLWYMKMMWAWLQAKRKPRKAPSRNICYDAFVSYSERDAYWVENLMVQELENFNPPFKLCLHKRDFIPGKWIIDNIIDSIEKSHKTVFVLSENFVKSEWCKYELDFSHFRLFDENNDAAILILLEPIEKKAIPQRFCKLRKIMNTKTYLEWPMDEAQREGFWVNLRAAIKSYFLGRLVPRGRGAAEAATRKQRITETESPYQELQGQRSDVYSDLNTQRPYYK

SEQ ID NO: 150 - protein, 749 aa, Artificial Sequence
  CER123 protein
  sig_peptide 1...22
MSKGLLLLWLVTELWWLYLTPAASEDTIIGFLGQPVTLPCHYLSWSQSRNSMCWGKGSCPNSKCNAELLRTDGTRIISRKSTKYTLLGKVQFGEVSLTISNTNRGDSGVYCCRIEVPGWFNDVKKNVRLELRRATTTKKPTTTTRPTTTPYVTTTTPELLPTTVMTTSVLPTTTPPQTLATTAFSTAVTTCPSTTPGSFSQETTKGSAFTTESETLPASNHSQRSMMTISTDIAVLRPTGSNPGILPSTSQLTTQKTTLTTSESLQKTTKSHQINSRQTILIIACCVGFVLMVLLFLAFLHRFHGLWYMKMMWAWLQAKRKPRKAPSRNICYDAFVSYSERDAYWVENLMVQELENFNPPFKLCLHKRDFIPGKWIIDNIIDSIEKSHKTVFVLSENFVKSEWCKYELDFSHFRLFDENNDAAILILLEPIEKKAIPQRFCKLRKIMNTKTYLEWPMDEAQREGFWVNLRAAIKSMSLLNCENSCGSSQSESDCCVAMASSCSAVTKDDSVGGTASTGNLSSSFMEEIQGYDVEFDPPLESKYECPICLMALREAVQTPCGHRFCKACIIKSIRDAGHKCPVDNEILLENQLFPDNFAKREILSLMVKCPNEGCLHKMELRHLEDHQAHCEFALMDCPQCQRPFQKFHINIHILKDCPRRQVSCDNCAASMAFEDKEIHDQNCPLANVICEYCNTILIREQMPNHYDLDCPTAPIPCTFSTFGCHEKMQRNHLARHLQENTQSHMRMLA

SEQ ID NO: 151 - protein, 561 aa, Artificial Sequence
  CER124 protein
  sig_peptide 1...22
MSKGLLLLWLVTELWWLYLTPAASEDTIIGFLGQPVTLPCHYLSWSQSRNSMCWGKGSCPNSKCNAELLRTDGTRIISRKSTKYTLLGKVQFGEVSLTISNTNRGDSGVYCCRIEVPGWFNDVKKNVRLELRRATTTKKPTTTTRPTTTPYVTTTTPELLPTTVMTTSVLPTTTPPQTLATTAFSTAVTTCPSTTPGSFSQETTKGSAFTTESETLPASNHSQRSMMTISTDIAVLRPTGSNPGILPSTSQLTTQKTTLTTSESLQKTTKSHQINSRQTILIIACCVGFVLMVLLFLAFLHRFHGLWYMKMMWAWLQAKRKPRKAPSRNICYDAFVSYSERDAYWVENLMVQELENFNPPFKLCLHKRDFIPGKWIIDNIIDSIEKSHKTVFVLSENFVKSEWCKYELDFSHFRLFDENNDAAILILLEPIEKKAIPQRFCKLRKIMNTKTYLEWPMDEAQREGFWVNLRAAIKSLWNKKRMRGPGKDPTRKCPDPRSASSPKQHPSESVYTALQRRETEVYACIENEDGSSPTAKQSPLSQERPHRFEDDGELNLVYENL

SEQ ID NO: 152 - protein, 520 aa, Artificial Sequence
  CER125A protein
  sig_peptide 1...22
MSKGLLLLWLVTELWWLYLTPAASEDTIIGFLGQPVTLPCHYLSWSQSRNSMCWGKGSCPNSKCNAELLRTDGTRIISRKSTKYTLLGKVQFGEVSLTISNTNRGDSGVYCCRIEVPGWFNDVKKNVRLELRRATTTKKPTTTTRPTTTPYVTTTTPELLPTTVMTTSVLPTTTPPQTLATTAFSTAVTTCPSTTPGSFSQETTKGSAFTTESETLPASNHSQRSMMTISTDIAVLRPTGSNPGILPSTSQLTTQKTTLTTSESLQKTTKSHQINSRQTILIIACCVGFVLMVLLFLAFLHRFHGLWYMKMMWAWLQAKRKPRKAPSRNICYDAFVSYSERDAYWVENLMVQELENFNPPFKLCLHKRDFIPGKWIIDNIIDSIEKSHKTVFVLSENFVKSEWCKYELDFSHFRLFDENNDAAILILLEPIEKKAIPQRFCKLRKIMNTKTYLEWPMDEAQREGFWVNLRAAIKSDSKAGMEEDHTYEGLDIDQTATYEDIVTLRTGEVKWSVGEHPGQE

SEQ ID NO: 153 - protein, 504 aa, Artificial Sequence
  CER125B protein
  sig_peptide 1...22
MSKGLLLLWLVTELWWLYLTPAASEDTIIGFLGQPVTLPCHYLSWSQSRNSMCWGKGSCPNSKCNAELLRTDGTRIISRKSTKYTLLGKVQFGEVSLTISNTNRGDSGVYCCRIEVPGWFNDVKKNVRLELRRATTTKKPTTTTRPTTTPYVTTTTPELLPTTVMTTSVLPTTTPPQTLATTAFSTAVTTCPSTTPGSFSQETTKGSAFTTESETLPASNHSQRSMMTISTDIAVLRPTGSNPGILPSTSQLTTQKTTLTTSESLQKTTKSHQINSRQTILIIACCVGFVLMVLLFLAFLHRFHGLWYMKMMWAWLQAKRKPRKAPSRNICYDAFVSYSERDAYWVENLMVQELENFNPPFKLCLHKRDFIPGKWIIDNIIDSIEKSHKTVFVLSENFVKSEWCKYELDFSHFRLFDENNDAAILILLEPIEKKAIPQRFCKLRKIMNTKTYLEWPMDEAQREGFWVNLRAAIKSDSKAGMEEDHTYEGLDIDQTATYEDIVTL

SEQ ID NO: 154 - protein, 24 aa, Artificial Sequence
  T2A self-cleaving peptide variant
LEGGGEGRGSLLTCGDVEENPGPR

SEQ ID NO: 155 - protein, 19 aa, Artificial Sequence
  T2A self-cleaving peptide variant
EGRGSLLTCGDVEENPGPR

SEQ ID NO: 156 - protein, 23 aa, Artificial Sequence
  T2A self-cleaving peptide variant
LEGGGEGRGSLLTCGDVEENPGP

SEQ ID NO: 157 - protein, 27 aa, Artificial Sequence
  P2A self-cleaving peptide variant
RAKRSGSGATNFSLLKQAGDVEENPGP

SEQ ID NO: 158 - protein, 598 aa, Artificial Sequence
  HPV16 E7 TCRbeta chain-P2A-TCRalpha chain
MAPGLLCWALLCLLGAGLVDAGVTQSPTHLIKTRGQQVTLRCSPKSGHDTVSWYQQALGQGPQFIFQYYEEEERQRGNFPDRFSGHQFPNYSSELNVNALLLGDSALYLCASSLGWRGGRYNEQFFGPGTRLTVLEDLRNVTPPKVSLFEPSKAEIANKQKATLVCLARGFFPDHVELSWWVNGKEVHSGVCTDPQAYKESNYSYCLSSRLRVSATFWHNPRNHFRCQVQFHGLSEEDKWPEGSPKPVTQNISAEAWGRADCGITSASYQQGVLSATILYEILLGKATLYAVLVSTLVVMAMVKRKNSRAKRSGSGATNFSLLKQAGDVEENPGPMWGVFLLYVSMKMGGTTGQNIDQPTEMTATEGAIVQINCTYQTSGFNGLFWYQQHAGEAPTFLSYNVLDGLEEKGRFSSFLSRSKGYSYLLLKELQMKDSASYLCASVDGNNRLAFGKGNQVVVIPNIQNPEPAVYQLKDPRSQDSTLCLFTDFDSQINVPKTMESGTFITDKCVLDMKAMDSKSNGAIAWSNQTSFTCQDIFKETNATYPSSDVPCDATLTEKSFETDMNLNFQNLLVIVLRILLLKVAGFNLLMTLRLWSS

SEQ ID NO: 159 - protein, 386 aa, Artificial Sequence
  CER25 protein
  sig_peptide 1...22
MSKGLLLLWLVTELWWLYLTPAASEDTIIGFLGQPVTLPCHYLSWSQSRNSMCWGKGSCPNSKCNAELLRTDGTRIISRKSTKYTLLGKVQFGEVSLTISNTNRGDSGVYCCRIEVPGWFNDVKKNVRLELRRATTTKKPTTTTRPTTTPYVTTTTPELLPTTVMTTSVLPTTTPPQTLATTAFSTAVTTCPSTTPGSFSQETTKGSAFTTESETLPASNHSQRSMMTISTDIAVLRPTGSNPGILPSTSQLTTQKTTLTTSESLQKTTKSHQINSRQTILIIACCVGFVLMVLLFLAFLLWNKKRMRGPGKDPTRKCPDPRSASSPKQHPSESVYTALQRRETEVYACIENEDGSSPTAKQSPLSQERPHRFEDDGELNLVYENL

SEQ ID NO: 160 - protein, 135 aa, Artificial Sequence
  HPV16 E7 TCR Vbeta region
MAPGLLCWALLCLLGAGLVDAGVTQSPTHLIKTRGQQVTLRCSPKSGHDTVSWYQQALGQGPQFIFQYYEEEERQRGNFPDRFSGHQFPNYSSELNVNALLLGDSALYLCASSLGWRGGRYNEQFFGPGTRLTVL

SEQ ID NO: 161 - protein, 173 aa, Artificial Sequence
  TCR Cbeta region, Cys-substituted
EDLRNVTPPKVSLFEPSKAEIANKQKATLVCLARGFFPDHVELSWWVNGKEVHSGVCTDPQAYKESNYSYCLSSRLRVSATFWHNPRNHFRCQVQFHGLSEEDKWPEGSPKPVTQNISAEAWGRADCGITSASYQQGVLSATILYEILLGKATLYAVLVSTLVVMAMVKRKNS

SEQ ID NO: 162 - protein, 126 aa, Artificial Sequence
  HPV16 E7TCR Valpha region
MWGVFLLYVSMKMGGTTGQNIDQPTEMTATEGAIVQINCTYQTSGFNGLFWYQQHAGEAPTFLSYNVLDGLEEKGRFSSFLSRSKGYSYLLLKELQMKDSASYLCASVDGNNRLAFGKGNQVVVIP

SEQ ID NO: 163 - protein, 137 aa, Artificial Sequence
  TCR Calpha region, Cys-substituted, LVL substituted
NIQNPEPAVYQLKDPRSQDSTLCLFTDFDSQINVPKTMESGTFITDKCVLDMKAMDSKSNGAIAWSNQTSFTCQDIFKETNATYPSSDVPCDATLTEKSFETDMNLNFQNLLVIVLRILLLKVAGFNLLMTLRLWSS

SEQ ID NO: 164 - protein, 1108 aa, Artificial Sequence
  CER5_T2A_HPV16_E7_TCR tandem cassette
MSKGLLLLWLVTELWWLYLTPAASEDTIIGFLGQPVTLPCHYLSWSQSRNSMCWGKGSCPNSKCNAELLRTDGTRIISRKSTKYTLLGKVQFGEVSLTISNTNRGDSGVYCCRIEVPGWFNDVKKNVRLELRRATTTKKPTTTTRPTTTPYVTTTTPELLPTTVMTTSVLPTTTPPQTLATTAFSTAVTTCPSTTPGSFSQETTKGSAFTTESETLPASNHSQRSMMTISTDIAVLRPTGSNPGILPSTSQLTTQKTTLTTSESLQKTTKSHQINSRQTILIIACCVGFVLMVLLFLAFLKFYFHLMLLAGCIKYGRGENIYDAFVIYSSQDEDWVRNELVKNLEEGVPPFQLCLHYRDFIPGVAIAANIIHEGFHKSRKVIVVVSQHFIQSRWCIFEYEIAQTWQFLSSRAGIIFIVLQKVEKTLLRQQVELYRLLSRNTYLEWEDSVLGRHIFWRRLRKALLDGKSWNPEGTVGTGCNWQEATSILEGGGEGRGSLLTCGDVEENPGPMAPGLLCWALLCLLGAGLVDAGVTQSPTHLIKTRGQQVTLRCSPKSGHDTVSWYQQALGQGPQFIFQYYEEEERQRGNFPDRFSGHQFPNYSSELNVNALLLGDSALYLCASSLGWRGGRYNEQFFGPGTRLTVLEDLRNVTPPKVSLFEPSKAEIANKQKATLVCLARGFFPDHVELSWWVNGKEVHSGVCTDPQAYKESNYSYCLSSRLRVSATFWHNPRNHFRCQVQFHGLSEEDKWPEGSPKPVTQNISAEAWGRADCGITSASYQQGVLSATILYEILLGKATLYAVLVSTLVVMAMVKRKNSRAKRSGSGATNFSLLKQAGDVEENPGPMWGVFLLYVSMKMGGTTGQNIDQPTEMTATEGAIVQINCTYQTSGFNGLFWYQQHAGEAPTFLSYNVLDGLEEKGRFSSFLSRSKGYSYLLLKELQMKDSASYLCASVDGNNRLAFGKGNQVVVIPNIQNPEPAVYQLKDPRSQDSTLCLFTDFDSQINVPKTMESGTFITDKCVLDMKAMDSKSNGAIAWSNQTSFTCQDIFKETNATYPSSDVPCDATLTEKSFETDMNLNFQNLLVIVLRILLLKVAGFNLLMTLRLWSS

SEQ ID NO: 165 - protein, 1119 aa, Artificial Sequence
  CER19_T2A_HPV16_E7_TCR tandem cassette
MSKGLLLLWLVTELWWLYLTPAASEDTIIGFLGQPVTLPCHYLSWSQSRNSMCWGKGSCPNSKCNAELLRTDGTRIISRKSTKYTLLGKVQFGEVSLTISNTNRGDSGVYCCRIEVPGWFNDVKKNVRLELRRATTTKKPTTTTRPTTTPYVTTTTPELLPTTVMTTSVLPTTTPPQTLATTAFSTAVTTCPSTTPGSFSQETTKGSAFTTESETLPASNHSQRSMMTISTDIAVLRPTGSNPGILPSTSQLTTQKTTLTTSESLQKTTKSHQINSRQTILIIACCVGFVLMVLLFLAFLTKFRGFCFICYKTAQRLVFKDHPQGTEPDMYKYDAYLCFSSKDFTWVQNALLKHLDTQYSDQNRFNLCFEERDFVPGENRIANIQDAIWNSRKIVCLVSRHFLRDGWCLEAFSYAQGRCLSDLNSALIMVVVGSLSQYQLMKHQSIRGFVQKQQYLRWPEDFQDVGWFLHKLSQQILKKEKEKKKDNNIPLQTVATISLEGGGEGRGSLLTCGDVEENPGPMAPGLLCWALLCLLGAGLVDAGVTQSPTHLIKTRGQQVTLRCSPKSGHDTVSWYQQALGQGPQFIFQYYEEEERQRGNFPDRFSGHQFPNYSSELNVNALLLGDSALYLCASSLGWRGGRYNEQFFGPGTRLTVLEDLRNVTPPKVSLFEPSKAEIANKQKATLVCLARGFFPDHVELSWWVNGKEVHSGVCTDPQAYKESNYSYCLSSRLRVSATFWHNPRNHFRCQVQFHGLSEEDKWPEGSPKPVTQNISAEAWGRADCGITSASYQQGVLSATILYEILLGKATLYAVLVSTLVVMAMVKRKNSRAKRSGSGATNFSLLKQAGDVEENPGPMWGVFLLYVSMKMGGTTGQNIDQPTEMTATEGAIVQINCTYQTSGFNGLFWYQQHAGEAPTFLSYNVLDGLEEKGRFSSFLSRSKGYSYLLLKELQMKDSASYLCASVDGNNRLAFGKGNQVVVIPNIQNPEPAVYQLKDPRSQDSTLCLFTDFDSQINVPKTMESGTFITDKCVLDMKAMDSKSNGAIAWSNQTSFTCQDIFKETNATYPSSDVPCDATLTEKSFETDMNLNFQNLLVIVLRILLLKVAGFNLLMTLRLWSS

SEQ ID NO: 166 - protein, 1114 aa, Artificial Sequence
  CER21_T2A_HPV16_E7_TCR tandem cassette
MSKGLLLLWLVTELWWLYLTPAASEDTIIGFLGQPVTLPCHYLSWSQSRNSMCWGKGSCPNSKCNAELLRTDGTRIISRKSTKYTLLGKVQFGEVSLTISNTNRGDSGVYCCRIEVPGWFNDVKKNVRLELRRATTTKKPTTTTRPTTTPYVTTTTPELLPTTVMTTSVLPTTTPPQTLATTAFSTAVTTCPSTTPGSFSQETTKGSAFTTESETLPASNHSQRSMMTISTDIAVLRPTGSNPGILPSTSQLTTQKTTLTTSESLQKTTKSHQINSRQTILIIACCVGFVLMVLLFLAFLHHLFYWDVWFIYNVCLAKVKGYRSLSTSQTFYDAYISYDTKDASVTDWVINELRYHLEESRDKNVLLCLEERDWDPGLAIIDNLMQSINQSKKTVFVLTKKYAKSWNFKTAFYLALQRLMDENMDVIIFILLEPVLQHSQYLRLRQRICKSSILQWPDNPKAEGLFWQTLRNVVLTENDSRYNNMYVDSIKQYLEGGGEGRGSLLTCGDVEENPGPMAPGLLCWALLCLLGAGLVDAGVTQSPTHLIKTRGQQVTLRCSPKSGHDTVSWYQQALGQGPQFIFQYYEEEERQRGNFPDRFSGHQFPNYSSELNVNALLLGDSALYLCASSLGWRGGRYNEQFFGPGTRLTVLEDLRNVTPPKVSLFEPSKAEIANKQKATLVCLARGFFPDHVELSWWVNGKEVHSGVCTDPQAYKESNYSYCLSSRLRVSATFWHNPRNHFRCQVQFHGLSEEDKWPEGSPKPVTQNISAEAWGRADCGITSASYQQGVLSATILYEILLGKATLYAVLVSTLVVMAMVKRKNSRAKRSGSGATNFSLLKQAGDVEENPGPMWGVFLLYVSMKMGGTTGQNIDQPTEMTATEGAIVQINCTYQTSGFNGLFWYQQHAGEAPTFLSYNVLDGLEEKGRFSSFLSRSKGYSYLLLKELQMKDSASYLCASVDGNNRLAFGKGNQVVVIPNIQNPEPAVYQLKDPRSQDSTLCLFTDFDSQINVPKTMESGTFITDKCVLDMKAMDSKSNGAIAWSNQTSFTCQDIFKETNATYPSSDVPCDATLTEKSFETDMNLNFQNLLVIVLRILLLKVAGFNLLMTLRLWSS

SEQ ID NO: 167 - protein, 1007 aa, Artificial Sequence
  CER25_T2A_HPV16_E7_TCR tandem cassette
MSKGLLLLWLVTELWWLYLTPAASEDTIIGFLGQPVTLPCHYLSWSQSRNSMCWGKGSCPNSKCNAELLRTDGTRIISRKSTKYTLLGKVQFGEVSLTISNTNRGDSGVYCCRIEVPGWFNDVKKNVRLELRRATTTKKPTTTTRPTTTPYVTTTTPELLPTTVMTTSVLPTTTPPQTLATTAFSTAVTTCPSTTPGSFSQETTKGSAFTTESETLPASNHSQRSMMTISTDIAVLRPTGSNPGILPSTSQLTTQKTTLTTSESLQKTTKSHQINSRQTILIIACCVGFVLMVLLFLAFLLWNKKRMRGPGKDPTRKCPDPRSASSPKQHPSESVYTALQRRETEVYACIENEDGSSPTAKQSPLSQERPHRFEDDGELNLVYENLLEGGGEGRGSLLTCGDVEENPGPMAPGLLCWALLCLLGAGLVDAGVTQSPTHLIKTRGQQVTLRCSPKSGHDTVSWYQQALGQGPQFIFQYYEEEERQRGNFPDRFSGHQFPNYSSELNVNALLLGDSALYLCASSLGWRGGRYNEQFFGPGTRLTVLEDLRNVTPPKVSLFEPSKAEIANKQKATLVCLARGFFPDHVELSWWVNGKEVHSGVCTDPQAYKESNYSYCLSSRLRVSATFWHNPRNHFRCQVQFHGLSEEDKWPEGSPKPVTQNISAEAWGRADCGITSASYQQGVLSATILYEILLGKATLYAVLVSTLVVMAMVKRKNSRAKRSGSGATNFSLLKQAGDVEENPGPMWGVFLLYVSMKMGGTTGQNIDQPTEMTATEGAIVQINCTYQTSGFNGLFWYQQHAGEAPTFLSYNVLDGLEEKGRFSSFLSRSKGYSYLLLKELQMKDSASYLCASVDGNNRLAFGKGNQVVVIPNIQNPEPAVYQLKDPRSQDSTLCLFTDFDSQINVPKTMESGTFITDKCVLDMKAMDSKSNGAIAWSNQTSFTCQDIFKETNATYPSSDVPCDATLTEKSFETDMNLNFQNLLVIVLRILLLKVAGFNLLMTLRLWSS

SEQ ID NO: 168 - protein, 1096 aa, Artificial Sequence
  CER27_T2A_HPV16_E7_TCR tandem cassette
MSKGLLLLWLVTELWWLYLTPAASEDTIIGFLGQPVTLPCHYLSWSQSRNSMCWGKGSCPNSKCNAELLRTDGTRIISRKSTKYTLLGKVQFGEVSLTISNTNRGDSGVYCCRIEVPGWFNDVKKNVRLELRRATTTKKPTTTTRPTTTPYVTTTTPELLPTTVMTTSVLPTTTPPQTLATTAFSTAVTTCPSTTPGSFSQETTKGSAFTTESETLPASNHSQRSMMTISTDIAVLRPTGSNPGILPSTSQLTTQKTTLTTSESLQKTTKSHQINSRQTILIIACCVGFVLMVLLFLAFLHRFHGLWYMKMMWAWLQAKRKPRKAPSRNICYDAFVSYSERDAYWVENLMVQELENFNPPFKLCLHKRDFIPGKWIIDNIIDSIEKSHKTVFVLSENFVKSEWCKYELDFSHFRLFDENNDAAILILLEPIEKKAIPQRFCKLRKIMNTKTYLEWPMDEAQREGFWVNLRAAIKSLEGGGEGRGSLLTCGDVEENPGPMAPGLLCWALLCLLGAGLVDAGVTQSPTHLIKTRGQQVTLRCSPKSGHDTVSWYQQALGQGPQFIFQYYEEEERQRGNFPDRFSGHQFPNYSSELNVNALLLGDSALYLCASSLGWRGGRYNEQFFGPGTRLTVLEDLRNVTPPKVSLFEPSKAEIANKQKATLVCLARGFFPDHVELSWWVNGKEVHSGVCTDPQAYKESNYSYCLSSRLRVSATFWHNPRNHFRCQVQFHGLSEEDKWPEGSPKPVTQNISAEAWGRADCGITSASYQQGVLSATILYEILLGKATLYAVLVSTLVVMAMVKRKNSRAKRSGSGATNFSLLKQAGDVEENPGPMWGVFLLYVSMKMGGTTGQNIDQPTEMTATEGAIVQINCTYQTSGFNGLFWYQQHAGEAPTFLSYNVLDGLEEKGRFSSFLSRSKGYSYLLLKELQMKDSASYLCASVDGNNRLAFGKGNQVVVIPNIQNPEPAVYQLKDPRSQDSTLCLFTDFDSQINVPKTMESGTFITDKCVLDMKAMDSKSNGAIAWSNQTSFTCQDIFKETNATYPSSDVPCDATLTEKSFETDMNLNFQNLLVIVLRILLLKVAGFNLLMTLRLWSS

SEQ ID NO: 169 - protein, 1195 aa, Artificial Sequence
  CER29_T2A_HPV16_E7_TCR tandem cassette
MSKGLLLLWLVTELWWLYLTPAASEDTIIGFLGQPVTLPCHYLSWSQSRNSMCWGKGSCPNSKCNAELLRTDGTRIISRKSTKYTLLGKVQFGEVSLTISNTNRGDSGVYCCRIEVPGWFNDVKKNVRLELRRATTTKKPTTTTRPTTTPYVTTTTPELLPTTVMTTSVLPTTTPPQTLATTAFSTAVTTCPSTTPGSFSQETTKGSAFTTESETLPASNHSQRSMMTISTDIAVLRPTGSNPGILPSTSQLTTQKTTLTTSESLQKTTKSHQINSRQTILIIACCVGFVLMVLLFLAFLMSLLNCENSCGSSQSESDCCVAMASSCSAVTKDDSVGGTASTGNLSSSFMEEIQGYDVEFDPPLESKYECPICLMALREAVQTPCGHRFCKACIIKSIRDAGHKCPVDNEILLENQLFPDNFAKREILSLMVKCPNEGCLHKMELRHLEDHQAHCEFALMDCPQCQRPFQKFHINIHILKDCPRRQVSCDNCAASMAFEDKEIHDQNCPLANVICEYCNTILIREQMPNHYDLDCPTAPIPCTFSTFGCHEKMQRNHLARHLQENTQSHMRMLALEGGGEGRGSLLTCGDVEENPGPMAPGLLCWALLCLLGAGLVDAGVTQSPTHLIKTRGQQVTLRCSPKSGHDTVSWYQQALGQGPQFIFQYYEEEERQRGNFPDRFSGHQFPNYSSELNVNALLLGDSALYLCASSLGWRGGRYNEQFFGPGTRLTVLEDLRNVTPPKVSLFEPSKAEIANKQKATLVCLARGFFPDHVELSWWVNGKEVHSGVCTDPQAYKESNYSYCLSSRLRVSATFWHNPRNHFRCQVQFHGLSEEDKWPEGSPKPVTQNISAEAWGRADCGITSASYQQGVLSATILYEILLGKATLYAVLVSTLVVMAMVKRKNSRAKRSGSGATNFSLLKQAGDVEENPGPMWGVFLLYVSMKMGGTTGQNIDQPTEMTATEGAIVQINCTYQTSGFNGLFWYQQHAGEAPTFLSYNVLDGLEEKGRFSSFLSRSKGYSYLLLKELQMKDSASYLCASVDGNNRLAFGKGNQVVVIPNIQNPEPAVYQLKDPRSQDSTLCLFTDFDSQINVPKTMESGTFITDKCVLDMKAMDSKSNGAIAWSNQTSFTCQDIFKETNATYPSSDVPCDATLTEKSFETDMNLNFQNLLVIVLRILLLKVAGFNLLMTLRLWSS

SEQ ID NO: 170 - protein, 1195 aa, Artificial Sequence
  CER31_T2A_HPV16_E7_TCR tandem cassette
MSKGLLLLWLVTELWWLYLTPAASEDTIIGFLGQPVTLPCHYLSWSQSRNSMCWGKGSCPNSKCNAELLRTDGTRIISRKSTKYTLLGKVQFGEVSLTISNTNRGDSGVYCCRIEVPGWFNDVKKNVRLELRRATTTKKPTTTTRPTTTPYVTTTTPELLPTTVMTTSVLPTTTPPQTLATTAFSTAVTTCPSTTPGSFSQETTKGSAFTTESETLPASNHSQRSMMTISTDIAVLRPTGSNPGILPSTSQLTTQKTTLTTSESLQKTTKSHQINSRQTILIIACCVGFVLMVLLFLAFLMESSKKMDSPGALQTNPPLKLHTDRSAGTPVFVPEQGGYKEKFVKTVEDKYKCEKCHLVLCSPKQTECGHRFCESCMAALLSSSSPKCTACQESIVKDKVFKDNCCKREILALQIYCRNESRGCAEQLMLGHLLVHLKNDCHFEELPCVRPDCKEKVLRKDLRDHVEKACKYREATCSHCKSQVPMIALQKHEDTDCPCVVVSCPHKCSVQTLLRSELSAHLSECVNAPSTCSFKRYGCVFQGTNQQIKAHEASSAVQHVNLLKEWSNSLEKKVLEGGGEGRGSLLTCGDVEENPGPMAPGLLCWALLCLLGAGLVDAGVTQSPTHLIKTRGQQVTLRCSPKSGHDTVSWYQQALGQGPQFIFQYYEEEERQRGNFPDRFSGHQFPNYSSELNVNALLLGDSALYLCASSLGWRGGRYNEQFFGPGTRLTVLEDLRNVTPPKVSLFEPSKAEIANKQKATLVCLARGFFPDHVELSWWVNGKEVHSGVCTDPQAYKESNYSYCLSSRLRVSATFWHNPRNHFRCQVQFHGLSEEDKWPEGSPKPVTQNISAEAWGRADCGITSASYQQGVLSATILYEILLGKATLYAVLVSTLVVMAMVKRKNSRAKRSGSGATNFSLLKQAGDVEENPGPMWGVFLLYVSMKMGGTTGQNIDQPTEMTATEGAIVQINCTYQTSGFNGLFWYQQHAGEAPTFLSYNVLDGLEEKGRFSSFLSRSKGYSYLLLKELQMKDSASYLCASVDGNNRLAFGKGNQVVVIPNIQNPEPAVYQLKDPRSQDSTLCLFTDFDSQINVPKTMESGTFITDKCVLDMKAMDSKSNGAIAWSNQTSFTCQDIFKETNATYPSSDVPCDATLTEKSFETDMNLNFQNLLVIVLRILLLKVAGFNLLMTLRLWSS

SEQ ID NO: 171 - protein, 155 aa, Homo sapiens
  truncated MyD88 signaling domain without TIR domain
MAAGGPGAGSAAPVSSTSSLPLAALNMRVRRRLSLFLNVRTQVAADWTALAEEMDFEYLEIRQLETQADPTGRLLDAWQGRPGASVGRLLELLTKLGRDDVLLELGPSIEEDCQKYILKQQQEEAEKPLQVAAVDSSVPRTAELAGITTLDDPLG

SEQ ID NO: 172 - protein, 296 aa, Homo sapiens
  MyD88 signaling domain
MAAGGPGAGSAAPVSSTSSLPLAALNMRVRRRLSLFLNVRTQVAADWTALAEEMDFEYLEIRQLETQADPTGRLLDAWQGRPGASVGRLLELLTKLGRDDVLLELGPSIEEDCQKYILKQQQEEAEKPLQVAAVDSSVPRTAELAGITTLDDPLGHMPERFDAFICYCPSDIQFVQEMIRQLEQTNYRLKLCVSDRDVLPGTCVWSIASELIEKRCRRMVVVVSDDYLQSKECDFQTKFALSLSPGAHQKRLIPIKYKAMKKEFPSILRFITVCDYTNPCTKSWFWTRLAKALSLP

SEQ ID NO: 173 - protein, 530 aa, Artificial Sequence
  CER119A protein
  sig_peptide 1...22
MSKGLLLLWLVTELWWLYLTPAASEDTIIGFLGQPVTLPCHYLSWSQSRNSMCWGKGSCPNSKCNAELLRTDGTRIISRKSTKYTLLGKVQFGEVSLTISNTNRGDSGVYCCRIEVPGWFNDVKKNVRLELRRATTTKKPTTTTRPTTTPYVTTTTPELLPTTVMTTSVLPTTTPPQTLATTAFSTAVTTCPSTTPGSFSQETTKGSAFTTESETLPASNHSQRSMMTISTDIAVLRPTGSNPGILPSTSQLTTQKTTLTTSESLQKTTKSHQINSRQTILIIACCVGFVLMVLLFLAFLSYLDLPWYLRMVCQWTQTRRRARNIPLEELQRNLQFHAFISYSGHDSFWVKNELLPNLEKEGMQICLHERNFVPGKSIVENIITCIEKSYKSIFVLSPNFVQSEWCHYELYFAHHNLFHEGSNSLILILLEPIPQYSIPSSYHKLKSLMARRTYLEWPKEKSKRGLFWANLRAAINIKLTEQAKKDSKAGMEEDHTYEGLDIDQTATYEDIVTLRTGEVKWSVGEHPGQE

SEQ ID NO: 174 - protein, 778 aa, Artificial Sequence
  CER126 protein
  sig_peptide 1...22
MSKGLLLLWLVTELWWLYLTPAASEDTIIGFLGQPVTLPCHYLSWSQSRNSMCWGKGSCPNSKCNAELLRTDGTRIISRKSTKYTLLGKVQFGEVSLTISNTNRGDSGVYCCRIEVPGWFNDVKKNVRLELRRATTTKKPTTTTRPTTTPYVTTTTPELLPTTVMTTSVLPTTTPPQTLATTAFSTAVTTCPSTTPGSFSQETTKGSAFTTESETLPASNHSQRSMMTISTDIAVLRPTGSNPGILPSTSQLTTQKTTLTTSESLQKTTKSHQINSRQTILIIACCVGFVLMVLLFLAFLHRFHGLWYMKMMWAWLQAKRKPRKAPSRNICYDAFVSYSERDAYWVENLMVQELENFNPPFKLCLHKRDFIPGKWIIDNIIDSIEKSHKTVFVLSENFVKSEWCKYELDFSHFRLFDENNDAAILILLEPIEKKAIPQRFCKLRKIMNTKTYLEWPMDEAQREGFWVNLRAAIKSMAAASVTPPGSLELLQPGFSKTLLGTKLEAKYLCSACRNVLRRPFQAQCGHRYCSFCLASILSSGPQNCAACVHEGIYEEGISILESSSAFPDNAARREVESLPAVCPSDGCTWKGTLKEYESCHEGRCPLMLTECPACKGLVRLGEKERHLEHECPERSLSCRHCRAPCCGADVKAHHEVCPKFPLTCDGCGKKKIPREKFQDHVKTCGKCRVPCRFHAIGCLETVEGEKQQEHEVQWLREHLAMLLSSVLEAKPLLGDQSHAGSELLQRCESLEKKTATFENIVCVLNREVERVAMTAEAC

SEQ ID NO: 175 - protein, 778 aa, Artificial Sequence
  CER127 protein
  sig_peptide 1...22
MSKGLLLLWLVTELWWLYLTPAASEDTIIGFLGQPVTLPCHYLSWSQSRNSMCWGKGSCPNSKCNAELLRTDGTRIISRKSTKYTLLGKVQFGEVSLTISNTNRGDSGVYCCRIEVPGWFNDVKKNVRLELRRATTTKKPTTTTRPTTTPYVTTTTPELLPTTVMTTSVLPTTTPPQTLATTAFSTAVTTCPSTTPGSFSQETTKGSAFTTESETLPASNHSQRSMMTISTDIAVLRPTGSNPGILPSTSQLTTQKTTLTTSESLQKTTKSHQINSRQTILIIACCVGFVLMVLLFLAFLMAAASVTPPGSLELLQPGFSKTLLGTKLEAKYLCSACRNVLRRPFQAQCGHRYCSFCLASILSSGPQNCAACVHEGIYEEGISILESSSAFPDNAARREVESLPAVCPSDGCTWKGTLKEYESCHEGRCPLMLTECPACKGLVRLGEKERHLEHECPERSLSCRHCRAPCCGADVKAHHEVCPKFPLTCDGCGKKKIPREKFQDHVKTCGKCRVPCRFHAIGCLETVEGEKQQEHEVQWLREHLAMLLSSVLEAKPLLGDQSHAGSELLQRCESLEKKTATFENIVCVLNREVERVAMTAEACHRFHGLWYMKMMWAWLQAKRKPRKAPSRNICYDAFVSYSERDAYWVENLMVQELENFNPPFKLCLHKRDFIPGKWIIDNIIDSIEKSHKTVFVLSENFVKSEWCKYELDFSHFRLFDENNDAAILILLEPIEKKAIPQRFCKLRKIMNTKTYLEWPMDEAQREGFWVNLRAAIKS

SEQ ID NO: 176 - protein, 796 aa, Artificial Sequence
  CER128 protein
  sig_peptide 1...22
MSKGLLLLWLVTELWWLYLTPAASEDTIIGFLGQPVTLPCHYLSWSQSRNSMCWGKGSCPNSKCNAELLRTDGTRIISRKSTKYTLLGKVQFGEVSLTISNTNRGDSGVYCCRIEVPGWFNDVKKNVRLELRRATTTKKPTTTTRPTTTPYVTTTTPELLPTTVMTTSVLPTTTPPQTLATTAFSTAVTTCPSTTPGSFSQETTKGSAFTTESETLPASNHSQRSMMTISTDIAVLRPTGSNPGILPSTSQLTTQKTTLTTSESLQKTTKSHQINSRQTILIIACCVGFVLMVLLFLAFLMAAASVTPPGSLELLQPGFSKTLLGTKLEAKYLCSACRNVLRRPFQAQCGHRYCSFCLASILSSGPQNCAACVHEGIYEEGISILESSSAFPDNAARREVESLPAVCPSDGCTWKGTLKEYESCHEGRCPLMLTECPACKGLVRLGEKERHLEHECPERSLSCRHCRAPCCGADVKAHHEVCPKFPLTCDGCGKKKIPREKFQDHVKTCGKCRVPCRFHAIGCLETVEGEKQQEHEVQWLREHLAMLLSSVLEAKPLLGDQSHAGSELLQRCESLEKKTATFENIVCVLNREVERVAMTAEACHHLFYWDVWFIYNVCLAKVKGYRSLSTSQTFYDAYISYDTKDASVTDWVINELRYHLEESRDKNVLLCLEERDWDPGLAIIDNLMQSINQSKKTVFVLTKKYAKSWNFKTAFYLALQRLMDENMDVIIFILLEPVLQHSQYLRLRQRICKSSILQWPDNPKAEGLFWQTLRNVVLTENDSRYNNMYVDSIKQY

SEQ ID NO: 177 - protein, 796 aa, Artificial Sequence
  CER129 protein
  sig_peptide 1...22
MSKGLLLLWLVTELWWLYLTPAASEDTIIGFLGQPVTLPCHYLSWSQSRNSMCWGKGSCPNSKCNAELLRTDGTRIISRKSTKYTLLGKVQFGEVSLTISNTNRGDSGVYCCRIEVPGWFNDVKKNVRLELRRATTTKKPTTTTRPTTTPYVTTTTPELLPTTVMTTSVLPTTTPPQTLATTAFSTAVTTCPSTTPGSFSQETTKGSAFTTESETLPASNHSQRSMMTISTDIAVLRPTGSNPGILPSTSQLTTQKTTLTTSESLQKTTKSHQINSRQTILIIACCVGFVLMVLLFLAFLHHLFYWDVWFIYNVCLAKVKGYRSLSTSQTFYDAYISYDTKDASVTDWVINELRYHLEESRDKNVLLCLEERDWDPGLAIIDNLMQSINQSKKTVFVLTKKYAKSWNFKTAFYLALQRLMDENMDVIIFILLEPVLQHSQYLRLRQRICKSSILQWPDNPKAEGLFWQTLRNVVLTENDSRYNNMYVDSIKQYMAAASVTPPGSLELLQPGFSKTLLGTKLEAKYLCSACRNVLRRPFQAQCGHRYCSFCLASILSSGPQNCAACVHEGIYEEGISILESSSAFPDNAARREVESLPAVCPSDGCTWKGTLKEYESCHEGRCPLMLTECPACKGLVRLGEKERHLEHECPERSLSCRHCRAPCCGADVKAHHEVCPKFPLTCDGCGKKKIPREKFQDHVKTCGKCRVPCRFHAIGCLETVEGEKQQEHEVQWLREHLAMLLSSVLEAKPLLGDQSHAGSELLQRCESLEKKTATFENIVCVLNREVERVAMTAEAC